European Patent Application EP 4 382 607 A1, published June 12, 2024. Title: Nucleic acid construct utilizing SNARE. Applicant: 花王株式会社. The sequence listing filed with the application follows.

SEQUENCE LISTING (98 sequences)

SEQ ID NO: 1 - DNA, 663 bp, Homo sapiens
  source 1..663: mol_type = genomic DNA
atggcgattctttttgctgttgttgccagggggaccactatccttgccaaacatgcttggtgtggaggaaacttcctggaggtgacagagcagattctggctaagataccttctgaaaataacaaactaacgtactcacatggcaattatttgtttcattacatctgccaagacaggattgtatatctttgtatcactgatgatgattttgaacgttcccgagcctttaattttctgaatgagataaagaagaggttccagactacttacggttcaagagcacagacagcacttccatatgccatgaatagcgagttctcaagtgtcttagctgcacagctgaagcatcactctgagaataagggcctagacaaagtgatggagactcaagcccaagtggatgaactgaaaggaatcatggtcagaaacatagatctggtagctcagcgaggagaaagattggaattattgattgacaaaacagaaaatcttgtggattcttctgtcaccttcaaaactaccagcagaaatcttgctcgagccatgtgtatgaagaacctcaagctcactattatcatcatcatcgtatcaattgtgttcatctatatcattgtttcacctctctgtggtggatttacatggccaagctgtgtgaagaaatag

SEQ ID NO: 2 - DNA, 774 bp, Homo sapiens
  source 1..774: mol_type = genomic DNA
atggatcccctgttccagcaaacgcacaagcaggtccacgagatccagtcttgcatgggacgcctggagacggcagacaagcagtctgtgcacatagtagaaaacgaaatccaagcaagcatagaccagatattcagccgtctagaacgtctggagattttgtccagcaaggagccccctaacaaaaggcaaaatgccagacttcgggttgaccagttaaagtatgatgtccagcacctgcagactgcgctcagaaacttccagcatcggcgccatgcaagggagcagcaggagagacagcgagaagagcttctgtctcgaaccttcaccactaacgactctgacaccaccataccaatggacgaatcactgcagtttaactcctccctccagaaagttcacaacggcatggatgacctcattttagatgggcacaatattttagatggactgaggacccagagactgaccttgaaggggactcagaagaagatccttgacattgccaacatgctgggcttgtccaacacagtgatgcggctcatcgagaagcgggctttccaggacaagtactttatgatagagacaaggtctcaccatgttgcccagaatggacccgaactcctgagctcaagagatcctcctgcatcagcctcccgaagtgctgggattataggtatgagccaccaccctgacctccaaataccttttgaactcaggcttggatttgaactctggttctatcaactattagctgtgatttcagatcagtga

SEQ ID NO: 3 - DNA, 750 bp, Homo sapiens
  source 1..750: mol_type = genomic DNA
atgtctctcgaagaccccttttttgtagtccgaggcgaggtgcagaaggcggtgaacacggcccgcgggctgtaccagcgctggtgcgagctcctgcaggaaagcgcggcggtcggacgcgaggagctggactggacgaccaatgagctgcggaatggcctgcgcagcatcgagtgggacctcgaggacctggaagagaccatcggtatagtggaagccaacccaggcaagttcaagctcccagccggggacctgcaggagagaaaggtgttcgtggagcggatgcgagaggcagtccaggaaatgaaggaccatatggtcagcccaacagccgtagcatttttggagaggaataacagagagatactcgcaggcaagccagctgcccagaagtcacccagcgacctgctggatgccagcgcagtctcggccacatctcgctacatcgaggagcagcaggccacacagcagctgatcatggatgaacaggatcaacagctggagatggtgtctgggagcatccaggttctgaagcacatgtccggccgcgttggagaagagctggacgagcagggcatcatgctggatgccttcgcccaagagatggaccacacccagtcccgcatggacggggtcctcaggaagttggccaaagtatcccacatgacgagtgaccgccgacagtggtgtgccatcgccgtgctagtgggggtgcttctcctcgttctcatcttactattctctctctga

SEQ ID NO: 4 - DNA, 1008 bp, Homo sapiens
  source 1..1008: mol_type = genomic DNA
atggcggtggacatcacgctgctattccgggccagcgtcaagaccgtgaagacgcggaacaaggcgctgggagtggcggtgggcggcggggtcgatggcagccgggacgagctgttccgccggagcccccggcccaagggcgacttctccagccgggcccgcgaagtgatttctcacattggcaaactgagagattttcttctggaacacaggaaagattatattaatgcttatagccataccatgtctgaatatgggaggatgacagacacagaacgagaccagatagaccaggatgcccagatattcatgaggacctgttcagaagcaattcagcaactacgaacagaagctcacaaggagatacattcccagcaagtgaaggagcacaggaccgctgttttggatttcattgaagattacttgaaaagagtatgtaaactttactcagaacagagagccatccgagttaaaagagtggtggataagaaaagattatctaagctggaaccagaaccaaatacaaagacaagagaatccacatcttctgagaaagtttcacagagtccttcaaaagactctgaagaaaaccctgccactgaagaacgtccagaaaaaattttggctgaaacacaacctgaattgggaacgtggggagatggcaaaggcgaagatgagttatccccagaagaaatacaaatgtttgaacaggaaaatcagcgactaattggtgaaatgaacagcttgtttgatgaagtgaggcaaatcgaagggagagtggttgagatttccagactccaagagatattcacggaaaaggttttgcaacaggaagctgagattgacagcattcaccagttagttgtgggggcaactgaaaatatcaaggaaggcaacgaagacataagagaggccattaaaaacaacgctggcttccgcgtgtggatcctcttcttcctcgtgatgtgctccttctccttgctcttcctcgactggtacgacagctag

SEQ ID NO: 5 - DNA, 816 bp, Homo sapiens
  source 1..816: mol_type = genomic DNA
atggcggctccccaagacgtccacgtccggatctgtaaccaagagattgtcaaatttgacctggaggtgaaggcgcttattcaggatatccgtgattgttcaggacccttaagtgctcttactgaactgaatactaaagtaaaagagaaatttcaacagttgcgtcacagaatacagccagttctctatcaaagggcatttatttggactgcttccacatttttttttaagctaacttattccctgacagacttttcttcaactcagcatgacttcaactctccaactacacctgttaccttcagtgacctggagcagttggctaaagagcaagacaaagaatcagagaaacaacttctactccaggaagtggagaatcacaaaaagcagatgctcagcaatcaggcctcatggaggaaagctaatctcacctgcaaaattgcaatcgacaatctagagaaagcagaacttcttcagggaggagatctcttaaggcaaaggaaaaccaccaaagagagcctggcccagacatccagtaccatcactgagagcctcatggggatcagcaggatgatggcccagcaggtccagcagagcgaggaggccatgcagtctctagtcacttcttcacgaacgatcctggatgcaaatgaagaatttaagtccatgtcgggcaccatccagctgggccggaagcttatcacaaaatacaatcgccgggagctgacggacaagcttctcatcttccttgcgctagccctgtttcttgctacggtcctctatattgtgaaaaagcggctctttccatttttgtga

SEQ ID NO: 6 - DNA, 786 bp, Homo sapiens
  source 1..786: mol_type = genomic DNA
atgtcttacactccaggagttggtggtgaccccgcccagttggcccagaggatctcttctaacatccagaagatcacacagtgttctgtggaaatacaaagaactctgaatcaacttggaacacctcaagattcacctgaattgaggcaacagttgcaacagaagcagcagtatactaaccagcttgccaaagaaacagataagtacattaaagagtttggatctctgcccaccacccccagtgaacagcgtcaaaggaaaatacagaaggatcgcttagtggcagagttcacaacatcactgacaaacttccagaaggtccagaggcaggctgctgagcgagagaaagagtttgttgctcgagtaagagccagttccagagtgtctggcagttttcctgaggacagctcaaaagaaaggaatcttgtatcctgggaaagccaaactcaacctcaagtgcaggtgcaggatgaagaaattacagaggatgacctccgtcttattcatgagagagaatcttctatcaggcaacttgaagctgatattatggatattaatgaaatatttaaagatttgggaatgatgattcatgaacaaggagatgtaatagatagcatagaagccaatgtggaaaatgcagaggtgcacgttcagcaagcaaatcagcagctgtcaagggcagcagattatcagcgcaaatccagaaaaaccctgtgcatcatcattcttatccttgtcattggagttgcgattatcagtctcatcatatggggattgaaccactga

SEQ ID NO: 7 - DNA, 675 bp, Homo sapiens
  source 1..675: mol_type = genomic DNA
atgtcgtccgacttcgaaggttacgagcaggacttcgcggtgctcactgcagagatcaccagcaagattgcgagggtcccacgactcccgcctgatgaaaagaaacagatggttgcaaatgtggagaaacagcttgaagaagcgaaagaactgcttgaacagatggatttggaagtccgagagataccaccccaaagtcgagggatgtacagcaacagaatgagaagctacaaacaagaaatgggaaaactcgaaacagattttaaaaggtcacggatcgcctacagtgacgaagtacggaatgagctcctgggggatgatgggaattcctcagagaaccagttgataaaattacgtgaagagagggcacatctgctcgataacacagagaggctggaaaggtcatctcggagactagaggctggataccaaatagcagtggaaaccgagcaaattggtcaggagatgttggaaaaccttagtcatgacagagaaaagatacagcgagcacgtgaaagacttcgggaaacagatgctaatttgggaaaaagctccaggattctgacagggatgttgcgaagaatcatccagaaccgcatcctgctcgtcatcctagggatcatcgtggtcatcaccatcctgatggcgatcactttttctgtcagaagacactga

SEQ ID NO: 8 - DNA, 978 bp, Homo sapiens
  source 1..978: mol_type = genomic DNA
atggccaccaggcgtttaaccgacgctttcttgttgttgcggaataattccatccaaaaccggcagctgttagccgagcaagtgagtagtcacatcacctccagccctctgcattcacgtagcattgctgcggagctggacgagcttgctgatgaccgtatggcactggtgtcaggcatcagcttagatccagaagcagcgattggtgtgacaaaacggccacctcctaagtgggtggatggagtggatgaaattcagtatgatgttggccggattaagcagaagatgaaagaattggccagccttcatgacaagcatttaaacagacccaccctggatgacagcagcgaagaggaacatgccattgagataactacccaagagatcactcagctcttccacaggtgccagcgtgccgtgcaggccctgccgagccgggcccgggcctgctccgagcaggaggggcggctgcttgggaacgtggtggcctcgctggcgcaggccctgcaggaactctccaccagcttccggcacgcacagtcaggctacctcaaacgcatgaagaatcgagaggaaagatcccagcattttttcgacacatcagtaccactaatggatgatggagacgataacactctttaccatcggggttttacagaggaccagttagttctggtggagcagaacacactgatggtggaagagcgggaacgagagattcgccagattgtacagtccatttctgacctgaatgaaatattcagggacttaggggcgatgattgtagaacagggtacagtccttgacagaattgactataacgttgaacagtcctgtatcaaaactgaagatggtttgaaacagcttcacaaggcagaacagtatcaaaagaagaatcggaagatgcttgtgattttaatattatttgtcatcatcattgtgctcattgttgtcctcgttggcgtgaagtctcgataa

SEQ ID NO: 9 - DNA, 1068 bp, Homo sapiens
  source 1..1068: mol_type = genomic DNA
atgatcccgcggaaacgctacgggtctaagaacacggatcagggtgtctacctgggtctctcaaagacacaggtcctgtcccctgcaactgctggcagtagcagcagcgacatcgcccctctgccccccccagtgaccctcgtccctccccctcccgacaccatgtcctgccgggatcggacccaggagtttctgtctgcctgcaagtcgctgcagacccgtcagaatggaatccagacaaataagccagctttgcgtgctgtccgacaacgcagtgaattcaccctcatggccaagcgcattgggaaagaccttagcaacacatttgccaagctggagaagctgacaatcttggcaaagcgcaagtccctctttgatgataaagcagtggaaattgaagagctaacatatatcatcaaacaggacatcaatagcctcaacaaacaaattgctcagctccaggatttcgtgagagccaagggcagccagagtggccggcacctgcagacccactccaacaccattgtggtctccttgcagtcgaaactggcttctatgtccaatgacttcaaatcggttttagaagtgaggacagagaacctgaagcagcagaggagccggagagagcagttctcccgggcacctgtgtcagccctgccccttgcccctaaccacctgggcggtggtgctgtggttctgggggcagagtcccatgcctccaaggatgtcgccatcgacatgatggactctcggaccagccagcagctgcagctcattgacgagcaggattcctacatccagagtcgggcagacaccatgcagaacattgagtcgacaattgttgagttgggctccatctttcagcagttggcacacatggttaaggaacaggaggaaaccattcagaggatcgacgagaacgtgctaggagcccagctggacgttgaggccgcccattcagagatcctcaagtacttccagtctgtcacctccaaccggtggctcatggtcaaaatcttcctcatcctcattgtcttcttcatcatctttgtggtcttccttgcttga

SEQ ID NO: 10 - protein, 220 aa, Homo sapiens
MAILFAVVARGTTILAKHAWCGGNFLEVTEQILAKIPSENNKLTYSHGNYLFHYICQDRIVYLCITDDDFERSRAFNFLNEIKKRFQTTYGSRAQTALPYAMNSEFSSVLAAQLKHHSENKGLDKVMETQAQVDELKGIMVRNIDLVAQRGERLELLIDKTENLVDSSVTFKTTSRNLARAMCMKNLKLTIIIIIVSIVFIYIIVSPLCGGFTWPSCVKK

SEQ ID NO: 11 - protein, 257 aa, Homo sapiens
MDPLFQQTHKQVHEIQSCMGRLETADKQSVHIVENEIQASIDQIFSRLERLEILSSKEPPNKRQNARLRVDQLKYDVQHLQTALRNFQHRRHAREQQERQREELLSRTFTTNDSDTTIPMDESLQFNSSLQKVHNGMDDLILDGHNILDGLRTQRLTLKGTQKKILDIANMLGLSNTVMRLIEKRAFQDKYFMIETRSHHVAQNGPELLSSRDPPASASRSAGIIGMSHHPDLQIPFELRLGFELWFYQLLAVISDQ

SEQ ID NO: 12 - protein, 249 aa, Homo sapiens
MSLEDPFFVVRGEVQKAVNTARGLYQRWCELLQESAAVGREELDWTTNELRNGLRSIEWDLEDLEETIGIVEANPGKFKLPAGDLQERKVFVERMREAVQEMKDHMVSPTAVAFLERNNREILAGKPAAQKSPSDLLDASAVSATSRYIEEQQATQQLIMDEQDQQLEMVSGSIQVLKHMSGRVGEELDEQGIMLDAFAQEMDHTQSRMDGVLRKLAKVSHMTSDRRQWCAIAVLVGVLLLVLILLFSL

SEQ ID NO: 13 - protein, 335 aa, Homo sapiens
MAVDITLLFRASVKTVKTRNKALGVAVGGGVDGSRDELFRRSPRPKGDFSSRAREVISHIGKLRDFLLEHRKDYINAYSHTMSEYGRMTDTERDQIDQDAQIFMRTCSEAIQQLRTEAHKEIHSQQVKEHRTAVLDFIEDYLKRVCKLYSEQRAIRVKRVVDKKRLSKLEPEPNTKTRESTSSEKVSQSPSKDSEENPATEERPEKILAETQPELGTWGDGKGEDELSPEEIQMFEQENQRLIGEMNSLFDEVRQIEGRVVEISRLQEIFTEKVLQQEAEIDSIHQLVVGATENIKEGNEDIREAIKNNAGFRVWILFFLVMCSFSLLFLDWYDS

SEQ ID NO: 14 - protein, 271 aa, Homo sapiens
MAAPQDVHVRICNQEIVKFDLEVKALIQDIRDCSGPLSALTELNTKVKEKFQQLRHRIQPVLYQRAFIWTASTFFFKLTYSLTDFSSTQHDFNSPTTPVTFSDLEQLAKEQDKESEKQLLLQEVENHKKQMLSNQASWRKANLTCKIAIDNLEKAELLQGGDLLRQRKTTKESLAQTSSTITESLMGISRMMAQQVQQSEEAMQSLVTSSRTILDANEEFKSMSGTIQLGRKLITKYNRRELTDKLLIFLALALFLATVLYIVKKRLFPFL

SEQ ID NO: 15 - protein, 261 aa, Homo sapiens
MSYTPGVGGDPAQLAQRISSNIQKITQCSVEIQRTLNQLGTPQDSPELRQQLQQKQQYTNQLAKETDKYIKEFGSLPTTPSEQRQRKIQKDRLVAEFTTSLTNFQKVQRQAAEREKEFVARVRASSRVSGSFPEDSSKERNLVSWESQTQPQVQVQDEEITEDDLRLIHERESSIRQLEADIMDINEIFKDLGMMIHEQGDVIDSIEANVENAEVHVQQANQQLSRAADYQRKSRKTLCIIILILVIGVAIISLIIWGLNH

SEQ ID NO: 16 - protein, 224 aa, Homo sapiens
MSSDFEGYEQDFAVLTAEITSKIARVPRLPPDEKKQMVANVEKQLEEAKELLEQMDLEVREIPPQSRGMYSNRMRSYKQEMGKLETDFKRSRIAYSDEVRNELLGDDGNSSENQLIKLREERAHLLDNTERLERSSRRLEAGYQIAVETEQIGQEMLENLSHDREKIQRARERLRETDANLGKSSRILTGMLRRIIQNRILLVILGIIVVITILMAITFSVRRH

SEQ ID NO: 17 - protein, 325 aa, Homo sapiens
MATRRLTDAFLLLRNNSIQNRQLLAEQVSSHITSSPLHSRSIAAELDELADDRMALVSGISLDPEAAIGVTKRPPPKWVDGVDEIQYDVGRIKQKMKELASLHDKHLNRPTLDDSSEEEHAIEITTQEITQLFHRCQRAVQALPSRARACSEQEGRLLGNVVASLAQALQELSTSFRHAQSGYLKRMKNREERSQHFFDTSVPLMDDGDDNTLYHRGFTEDQLVLVEQNTLMVEEREREIRQIVQSISDLNEIFRDLGAMIVEQGTVLDRIDYNVEQSCIKTEDGLKQLHKAEQYQKKNRKMLVILILFVIIIVLIVVLVGVKSR

SEQ ID NO: 18 - protein, 355 aa, Homo sapiens
MIPRKRYGSKNTDQGVYLGLSKTQVLSPATAGSSSSDIAPLPPPVTLVPPPPDTMSCRDRTQEFLSACKSLQTRQNGIQTNKPALRAVRQRSEFTLMAKRIGKDLSNTFAKLEKLTILAKRKSLFDDKAVEIEELTYIIKQDINSLNKQIAQLQDFVRAKGSQSGRHLQTHSNTIVVSLQSKLASMSNDFKSVLEVRTENLKQQRSRREQFSRAPVSALPLAPNHLGGGAVVLGAESHASKDVAIDMMDSRTSQQLQLIDEQDSYIQSRADTMQNIESTIVELGSIFQQLAHMVKEQEETIQRIDENVLGAQLDVEAAHSEILKYFQSVTSNRWLMVKIFLILIVFFIIFVVFLA

SEQ ID NO: 19 - DNA, 45 bp, synthetic construct
  source 1..45: mol_type = other DNA; note = linker
ggcggcggaggatctggcggaggtggaagcggaggcggaggaagt

SEQ ID NO: 20 - protein, 15 aa, synthetic construct
  source 1..15: note = linker
GGGGSGGGGSGGGGS

SEQ ID NO: 21 - DNA, 15 bp, synthetic construct
  source 1..15: mol_type = other DNA; note = proprotein convertase (e.g., furin) recognition sequence
agaagggccagaaga

SEQ ID NO: 22 - protein, 5 aa, synthetic construct
  source 1..5: note = proprotein convertase (e.g., furin) recognition sequence
RRARR

SEQ ID NO: 23 - DNA, 1161 bp, Gallus gallus
  source 1..1161: mol_type = genomic DNA
atgggctccatcggcgcagcaagcatggaattttgttttgatgtattcaaggagctcaaagtccaccatgccaatgagaacatcttctactgccccattgccatcatgtcagctctagccatggtatacctgggtgcaaaagacagcaccaggacacagataaataaggttgttcgctttgataaacttccaggattcggagacagtattgaagctcagtgtggcacatctgtaaacgttcactcttcacttagagacatcctcaaccaaatcaccaaaccaaatgatgtttattcgttcagccttgccagtagactttatgctgaagagagatacccaatcctgccagaatacttgcagtgtgtgaaggaactgtatagaggaggcttggaacctatcaactttcaaacagctgcagatcaagccagagagctcatcaattcctgggtagaaagtcagacaaatggaattatcagaaatgtccttcagccaagctccgtggattctcaaactgcaatggttctggttaatgccattgtcttcaaaggactgtgggagaaaacatttaaggatgaagacacacaagcaatgcctttcagagtgactgagcaagaaagcaaacctgtgcagatgatgtaccagattggtttatttagagtggcatcaatggcttctgagaaaatgaagatcctggagcttccatttgccagtgggacaatgagcatgttggtgctgttgcctgatgaagtctcaggccttgagcagcttgagagtataatcaactttgaaaaactgactgaatggaccagttctaatgttatggaagagaggaagatcaaagtgtacttacctcgcatgaagatggaggaaaaatacaacctcacatctgtcttaatggctatgggcattactgacgtgtttagctcttcagccaatctgtctggcatctcctcagcagagagcctgaagatatctcaagctgtccatgcagcacatgcagaaatcaatgaagcaggcagagaggtggtagggtcagcagaggctggagtggatgctgcaagcgtctctgaagaatttagggctgaccatccattcctcttctgtatcaagcacatcgcaaccaacgccgttctcttctttggcagatgtgtttccccttaa

SEQ ID NO: 24 - protein, 386 aa, Gallus gallus
MGSIGAASMEFCFDVFKELKVHHANENIFYCPIAIMSALAMVYLGAKDSTRTQINKVVRFDKLPGFGDSIEAQCGTSVNVHSSLRDILNQITKPNDVYSFSLASRLYAEERYPILPEYLQCVKELYRGGLEPINFQTAADQARELINSWVESQTNGIIRNVLQPSSVDSQTAMVLVNAIVFKGLWEKTFKDEDTQAMPFRVTEQESKPVQMMYQIGLFRVASMASEKMKILELPFASGTMSMLVLLPDEVSGLEQLESIINFEKLTEWTSSNVMEERKIKVYLPRMKMEEKYNLTSVLMAMGITDVFSSSANLSGISSAESLKISQAVHAAHAEINEAGREVVGSAEAGVDAASVSEEFRADHPFLFCIKHIATNAVLFFGRCVSP

SEQ ID NO: 25 - protein, 621 aa, synthetic construct
  source 1..621: note = VAMP7-OVA
MAILFAVVARGTTILAKHAWCGGNFLEVTEQILAKIPSENNKLTYSHGNYLFHYICQDRIVYLCITDDDFERSRAFNFLNEIKKRFQTTYGSRAQTALPYAMNSEFSSVLAAQLKHHSENKGLDKVMETQAQVDELKGIMVRNIDLVAQRGERLELLIDKTENLVDSSVTFKTTSRNLARAMCMKNLKLTIIIIIVSIVFIYIIVSPLCGGFTWPSCVKKSGGGGSGGGGSGGGGSGSIGAASMEFCFDVFKELKVHHANENIFYCPIAIMSALAMVYLGAKDSTRTQINKVVRFDKLPGFGDSIEAQCGTSVNVHSSLRDILNQITKPNDVYSFSLASRLYAEERYPILPEYLQCVKELYRGGLEPINFQTAADQARELINSWVESQTNGIIRNVLQPSSVDSQTAMVLVNAIVFKGLWEKTFKDEDTQAMPFRVTEQESKPVQMMYQIGLFRVASMASEKMKILELPFASGTMSMLVLLPDEVSGLEQLESIINFEKLTEWTSSNVMEERKIKVYLPRMKMEEKYNLTSVLMAMGITDVFSSSANLSGISSAESLKISQAVHAAHAEINEAGREVVGSAEAGVDAASVSEEFRADHPFLFCIKHIATNAVLFFGRCVSP

SEQ ID NO: 26 - protein, 657 aa, synthetic construct
  source 1..657: note = GOSR2-OVA
MDPLFQQTHKQVHEIQSCMGRLETADKQSVHIVENEIQASIDQIFSRLERLEILSSKEPPNKRQNARLRVDQLKYDVQHLQTALRNFQHRRHAREQQERQREELLSRTFTTNDSDTTIPMDESLQFNSSLQKVHNGMDDLILDGHNILDGLRTQRLTLKGTQKKILDIANMLGLSNTVMRLIEKRAFQDKYFMIETRSHHVAQNGPELLSSRDPPASASRSAGIIGMSHHPDLQIPFELRLGFELWFYQLLAVISDQGGGGSGGGGSGGGGSGSIGAASMEFCFDVFKELKVHHANENIFYCPIAIMSALAMVYLGAKDSTRTQINKVVRFDKLPGFGDSIEAQCGTSVNVHSSLRDILNQITKPNDVYSFSLASRLYAEERYPILPEYLQCVKELYRGGLEPINFQTAADQARELINSWVESQTNGIIRNVLQPSSVDSQTAMVLVNAIVFKGLWEKTFKDEDTQAMPFRVTEQESKPVQMMYQIGLFRVASMASEKMKILELPFASGTMSMLVLLPDEVSGLEQLESIINFEKLTEWTSSNVMEERKIKVYLPRMKMEEKYNLTSVLMAMGITDVFSSSANLSGISSAESLKISQAVHAAHAEINEAGREVVGSAEAGVDAASVSEEFRADHPFLFCIKHIATNAVLFFGRCVSP

SEQ ID NO: 27 - protein, 649 aa, synthetic construct
  source 1..649: note = STX10-OVA
MSLEDPFFVVRGEVQKAVNTARGLYQRWCELLQESAAVGREELDWTTNELRNGLRSIEWDLEDLEETIGIVEANPGKFKLPAGDLQERKVFVERMREAVQEMKDHMVSPTAVAFLERNNREILAGKPAAQKSPSDLLDASAVSATSRYIEEQQATQQLIMDEQDQQLEMVSGSIQVLKHMSGRVGEELDEQGIMLDAFAQEMDHTQSRMDGVLRKLAKVSHMTSDRRQWCAIAVLVGVLLLVLILLFSLGGGGSGGGGSGGGGSGSIGAASMEFCFDVFKELKVHHANENIFYCPIAIMSALAMVYLGAKDSTRTQINKVVRFDKLPGFGDSIEAQCGTSVNVHSSLRDILNQITKPNDVYSFSLASRLYAEERYPILPEYLQCVKELYRGGLEPINFQTAADQARELINSWVESQTNGIIRNVLQPSSVDSQTAMVLVNAIVFKGLWEKTFKDEDTQAMPFRVTEQESKPVQMMYQIGLFRVASMASEKMKILELPFASGTMSMLVLLPDEVSGLEQLESIINFEKLTEWTSSNVMEERKIKVYLPRMKMEEKYNLTSVLMAMGITDVFSSSANLSGISSAESLKISQAVHAAHAEINEAGREVVGSAEAGVDAASVSEEFRADHPFLFCIKHIATNAVLFFGRCVSP

SEQ ID NO: 28 - protein, 735 aa, synthetic construct
  source 1..735: note = STX18-OVA
MAVDITLLFRASVKTVKTRNKALGVAVGGGVDGSRDELFRRSPRPKGDFSSRAREVISHIGKLRDFLLEHRKDYINAYSHTMSEYGRMTDTERDQIDQDAQIFMRTCSEAIQQLRTEAHKEIHSQQVKEHRTAVLDFIEDYLKRVCKLYSEQRAIRVKRVVDKKRLSKLEPEPNTKTRESTSSEKVSQSPSKDSEENPATEERPEKILAETQPELGTWGDGKGEDELSPEEIQMFEQENQRLIGEMNSLFDEVRQIEGRVVEISRLQEIFTEKVLQQEAEIDSIHQLVVGATENIKEGNEDIREAIKNNAGFRVWILFFLVMCSFSLLFLDWYDSGGGGSGGGGSGGGGSGSIGAASMEFCFDVFKELKVHHANENIFYCPIAIMSALAMVYLGAKDSTRTQINKVVRFDKLPGFGDSIEAQCGTSVNVHSSLRDILNQITKPNDVYSFSLASRLYAEERYPILPEYLQCVKELYRGGLEPINFQTAADQARELINSWVESQTNGIIRNVLQPSSVDSQTAMVLVNAIVFKGLWEKTFKDEDTQAMPFRVTEQESKPVQMMYQIGLFRVASMASEKMKILELPFASGTMSMLVLLPDEVSGLEQLESIINFEKLTEWTSSNVMEERKIKVYLPRMKMEEKYNLTSVLMAMGITDVFSSSANLSGISSAESLKISQAVHAAHAEINEAGREVVGSAEAGVDAASVSEEFRADHPFLFCIKHIATNAVLFFGRCVSP

SEQ ID NO: 29 - protein, 671 aa, synthetic construct
  source 1..671: note = BNIP1-OVA
MAAPQDVHVRICNQEIVKFDLEVKALIQDIRDCSGPLSALTELNTKVKEKFQQLRHRIQPVLYQRAFIWTASTFFFKLTYSLTDFSSTQHDFNSPTTPVTFSDLEQLAKEQDKESEKQLLLQEVENHKKQMLSNQASWRKANLTCKIAIDNLEKAELLQGGDLLRQRKTTKESLAQTSSTITESLMGISRMMAQQVQQSEEAMQSLVTSSRTILDANEEFKSMSGTIQLGRKLITKYNRRELTDKLLIFLALALFLATVLYIVKKRLFPFLGGGGSGGGGSGGGGSGSIGAASMEFCFDVFKELKVHHANENIFYCPIAIMSALAMVYLGAKDSTRTQINKVVRFDKLPGFGDSIEAQCGTSVNVHSSLRDILNQITKPNDVYSFSLASRLYAEERYPILPEYLQCVKELYRGGLEPINFQTAADQARELINSWVESQTNGIIRNVLQPSSVDSQTAMVLVNAIVFKGLWEKTFKDEDTQAMPFRVTEQESKPVQMMYQIGLFRVASMASEKMKILELPFASGTMSMLVLLPDEVSGLEQLESIINFEKLTEWTSSNVMEERKIKVYLPRMKMEEKYNLTSVLMAMGITDVFSSSANLSGISSAESLKISQAVHAAHAEINEAGREVVGSAEAGVDAASVSEEFRADHPFLFCIKHIATNAVLFFGRCVSP

SEQ ID NO: 30 - protein, 661 aa, synthetic construct
  source 1..661: note = STX7-OVA
MSYTPGVGGDPAQLAQRISSNIQKITQCSVEIQRTLNQLGTPQDSPELRQQLQQKQQYTNQLAKETDKYIKEFGSLPTTPSEQRQRKIQKDRLVAEFTTSLTNFQKVQRQAAEREKEFVARVRASSRVSGSFPEDSSKERNLVSWESQTQPQVQVQDEEITEDDLRLIHERESSIRQLEADIMDINEIFKDLGMMIHEQGDVIDSIEANVENAEVHVQQANQQLSRAADYQRKSRKTLCIIILILVIGVAIISLIIWGLNHGGGGSGGGGSGGGGSGSIGAASMEFCFDVFKELKVHHANENIFYCPIAIMSALAMVYLGAKDSTRTQINKVVRFDKLPGFGDSIEAQCGTSVNVHSSLRDILNQITKPNDVYSFSLASRLYAEERYPILPEYLQCVKELYRGGLEPINFQTAADQARELINSWVESQTNGIIRNVLQPSSVDSQTAMVLVNAIVFKGLWEKTFKDEDTQAMPFRVTEQESKPVQMMYQIGLFRVASMASEKMKILELPFASGTMSMLVLLPDEVSGLEQLESIINFEKLTEWTSSNVMEERKIKVYLPRMKMEEKYNLTSVLMAMGITDVFSSSANLSGISSAESLKISQAVHAAHAEINEAGREVVGSAEAGVDAASVSEEFRADHPFLFCIKHIATNAVLFFGRCVSP

SEQ ID NO: 31 - protein, 624 aa, synthetic construct
  source 1..624: note = VTI1A-OVA
MSSDFEGYEQDFAVLTAEITSKIARVPRLPPDEKKQMVANVEKQLEEAKELLEQMDLEVREIPPQSRGMYSNRMRSYKQEMGKLETDFKRSRIAYSDEVRNELLGDDGNSSENQLIKLREERAHLLDNTERLERSSRRLEAGYQIAVETEQIGQEMLENLSHDREKIQRARERLRETDANLGKSSRILTGMLRRIIQNRILLVILGIIVVITILMAITFSVRRHGGGGSGGGGSGGGGSGSIGAASMEFCFDVFKELKVHHANENIFYCPIAIMSALAMVYLGAKDSTRTQINKVVRFDKLPGFGDSIEAQCGTSVNVHSSLRDILNQITKPNDVYSFSLASRLYAEERYPILPEYLQCVKELYRGGLEPINFQTAADQARELINSWVESQTNGIIRNVLQPSSVDSQTAMVLVNAIVFKGLWEKTFKDEDTQAMPFRVTEQESKPVQMMYQIGLFRVASMASEKMKILELPFASGTMSMLVLLPDEVSGLEQLESIINFEKLTEWTSSNVMEERKIKVYLPRMKMEEKYNLTSVLMAMGITDVFSSSANLSGISSAESLKISQAVHAAHAEINEAGREVVGSAEAGVDAASVSEEFRADHPFLFCIKHIATNAVLFFGRCVSP

SEQ ID NO: 32 - protein, 725 aa, synthetic construct
  source 1..725: note = STX16-OVA
MATRRLTDAFLLLRNNSIQNRQLLAEQVSSHITSSPLHSRSIAAELDELADDRMALVSGISLDPEAAIGVTKRPPPKWVDGVDEIQYDVGRIKQKMKELASLHDKHLNRPTLDDSSEEEHAIEITTQEITQLFHRCQRAVQALPSRARACSEQEGRLLGNVVASLAQALQELSTSFRHAQSGYLKRMKNREERSQHFFDTSVPLMDDGDDNTLYHRGFTEDQLVLVEQNTLMVEEREREIRQIVQSISDLNEIFRDLGAMIVEQGTVLDRIDYNVEQSCIKTEDGLKQLHKAEQYQKKNRKMLVILILFVIIIVLIVVLVGVKSRGGGGSGGGGSGGGGSGSIGAASMEFCFDVFKELKVHHANENIFYCPIAIMSALAMVYLGAKDSTRTQINKVVRFDKLPGFGDSIEAQCGTSVNVHSSLRDILNQITKPNDVYSFSLASRLYAEERYPILPEYLQCVKELYRGGLEPINFQTAADQARELINSWVESQTNGIIRNVLQPSSVDSQTAMVLVNAIVFKGLWEKTFKDEDTQAMPFRVTEQESKPVQMMYQIGLFRVASMASEKMKILELPFASGTMSMLVLLPDEVSGLEQLESIINFEKLTEWTSSNVMEERKIKVYLPRMKMEEKYNLTSVLMAMGITDVFSSSANLSGISSAESLKISQAVHAAHAEINEAGREVVGSAEAGVDAASVSEEFRADHPFLFCIKHIATNAVLFFGRCVSP

SEQ ID NO: 33 - protein, 755 aa, synthetic construct
  source 1..755: note = STX5-OVA
MIPRKRYGSKNTDQGVYLGLSKTQVLSPATAGSSSSDIAPLPPPVTLVPPPPDTMSCRDRTQEFLSACKSLQTRQNGIQTNKPALRAVRQRSEFTLMAKRIGKDLSNTFAKLEKLTILAKRKSLFDDKAVEIEELTYIIKQDINSLNKQIAQLQDFVRAKGSQSGRHLQTHSNTIVVSLQSKLASMSNDFKSVLEVRTENLKQQRSRREQFSRAPVSALPLAPNHLGGGAVVLGAESHASKDVAIDMMDSRTSQQLQLIDEQDSYIQSRADTMQNIESTIVELGSIFQQLAHMVKEQEETIQRIDENVLGAQLDVEAAHSEILKYFQSVTSNRWLMVKIFLILIVFFIIFVVFLAGGGGSGGGGSGGGGSGSIGAASMEFCFDVFKELKVHHANENIFYCPIAIMSALAMVYLGAKDSTRTQINKVVRFDKLPGFGDSIEAQCGTSVNVHSSLRDILNQITKPNDVYSFSLASRLYAEERYPILPEYLQCVKELYRGGLEPINFQTAADQARELINSWVESQTNGIIRNVLQPSSVDSQTAMVLVNAIVFKGLWEKTFKDEDTQAMPFRVTEQESKPVQMMYQIGLFRVASMASEKMKILELPFASGTMSMLVLLPDEVSGLEQLESIINFEKLTEWTSSNVMEERKIKVYLPRMKMEEKYNLTSVLMAMGITDVFSSSANLSGISSAESLKISQAVHAAHAEINEAGREVVGSAEAGVDAASVSEEFRADHPFLFCIKHIATNAVLFFGRCVSP

SEQ ID NO: 34 - protein, 655 aa, synthetic construct
  source 1..655: note = STX6-OVA
MSMEDPFFVVKGEVQKAVNTAQGLFQRWTELLQDPSTATREEIDWTTNELRNNLRSIEWDLEDLDETISIVEANPRKFNLDATELSIRKAFITSTRQVVRDMKDQMSTSSVQALAERKNRQALLGDSGSQNWSTGTTDKYGRLDRELQRANSHFIEEQQAQQQLIVEQQDEQLELVSGSIGVLKNMSQRIGGELEEQAVMLEDFSHELESTQSRLDNVMKKLAKVSHMTSDRRQWCAIAILFAVLLVVLILFLVLGGGGSGGGGSGGGGSGSIGAASMEFCFDVFKELKVHHANENIFYCPIAIMSALAMVYLGAKDSTRTQINKVVRFDKLPGFGDSIEAQCGTSVNVHSSLRDILNQITKPNDVYSFSLASRLYAEERYPILPEYLQCVKELYRGGLEPINFQTAADQARELINSWVESQTNGIIRNVLQPSSVDSQTAMVLVNAIVFKGLWEKTFKDEDTQAMPFRVTEQESKPVQMMYQIGLFRVASMASEKMKILELPFASGTMSMLVLLPDEVSGLEQLESIINFEKLTEWTSSNVMEERKIKVYLPRMKMEEKYNLTSVLMAMGITDVFSSSANLSGISSAESLKISQAVHAAHAEINEAGREVVGSAEAGVDAASVSEEFRADHPFLFCIKHIATNAVLFFGRCVSP

SEQ ID NO: 35 - protein, 636 aa, synthetic construct
  source 1..636: note = STX8-OVA
MAPDPWFSTYDSTCQIAQEIAEKIQQRNQYERKGEKAPKLTVTIRALLQNLKEKIALLKDLLLRAVSTHQITQLEGDRRQNLLDDLVTRERLLLASFKNEGAEPDLIRSSLMSEEAKRGAPNPWLFEEPEETRGLGFDEIRQQQQKIIQEQDAGLDALSSIISRQKQMGQEIGNELDEQNEIIDDLANLVENTDEKLRNETRRVNMVDRKSASCGMIMVILLLLVAIVVVAVWPTNGGGGSGGGGSGGGGSGSIGAASMEFCFDVFKELKVHHANENIFYCPIAIMSALAMVYLGAKDSTRTQINKVVRFDKLPGFGDSIEAQCGTSVNVHSSLRDILNQITKPNDVYSFSLASRLYAEERYPILPEYLQCVKELYRGGLEPINFQTAADQARELINSWVESQTNGIIRNVLQPSSVDSQTAMVLVNAIVFKGLWEKTFKDEDTQAMPFRVTEQESKPVQMMYQIGLFRVASMASEKMKILELPFASGTMSMLVLLPDEVSGLEQLESIINFEKLTEWTSSNVMEERKIKVYLPRMKMEEKYNLTSVLMAMGITDVFSSSANLSGISSAESLKISQAVHAAHAEINEAGREVVGSAEAGVDAASVSEEFRADHPFLFCIKHIATNAVLFFGRCVSP

SEQ ID NO: 36 - protein, 676 aa, synthetic construct
  source 1..676: note = STX12-OVA
MSYGPLDMYRNPGPSGPQLRDFSSIIQTCSGNIQRISQATAQIKNLMSQLGTKQDSSKLQENLQQLQHSTNQLAKETNELLKELGSLPLPLSTSEQRQQRLQKERLMNDFSAALNNFQAVQRRVSEKEKESIARARAGSRLSAEERQREEQLVSFDSHEEWNQMQSQEDEVAITEQDLELIKERETAIRQLEADILDVNQIFKDLAMMIHDQGDLIDSIEANVESSEVHVERATEQLQRAAYYQKKSRKKMCILVLVLSVIILILGLIIWLVYKTKGGGGSGGGGSGGGGSGSIGAASMEFCFDVFKELKVHHANENIFYCPIAIMSALAMVYLGAKDSTRTQINKVVRFDKLPGFGDSIEAQCGTSVNVHSSLRDILNQITKPNDVYSFSLASRLYAEERYPILPEYLQCVKELYRGGLEPINFQTAADQARELINSWVESQTNGIIRNVLQPSSVDSQTAMVLVNAIVFKGLWEKTFKDEDTQAMPFRVTEQESKPVQMMYQIGLFRVASMASEKMKILELPFASGTMSMLVLLPDEVSGLEQLESIINFEKLTEWTSSNVMEERKIKVYLPRMKMEEKYNLTSVLMAMGITDVFSSSANLSGISSAESLKISQAVHAAHAEINEAGREVVGSAEAGVDAASVSEEFRADHPFLFCIKHIATNAVLFFGRCVSP

SEQ ID NO: 37 - protein, 500 aa, synthetic construct
  source 1..500: note = VAMP3-OVA
MSTGPTAATGSNRRLQQTQNQVDEVVDIMRVNVDKVLERDQKLSELDDRADALQAGASQFETSAAKLKRKYWWKNCKMWAIGITVLVIFIIIIIVWVVSSGGGGSGGGGSGGGGSGSIGAASMEFCFDVFKELKVHHANENIFYCPIAIMSALAMVYLGAKDSTRTQINKVVRFDKLPGFGDSIEAQCGTSVNVHSSLRDILNQITKPNDVYSFSLASRLYAEERYPILPEYLQCVKELYRGGLEPINFQTAADQARELINSWVESQTNGIIRNVLQPSSVDSQTAMVLVNAIVFKGLWEKTFKDEDTQAMPFRVTEQESKPVQMMYQIGLFRVASMASEKMKILELPFASGTMSMLVLLPDEVSGLEQLESIINFEKLTEWTSSNVMEERKIKVYLPRMKMEEKYNLTSVLMAMGITDVFSSSANLSGISSAESLKISQAVHAAHAEINEAGREVVGSAEAGVDAASVSEEFRADHPFLFCIKHIATNAVLFFGRCVSP

SEQ ID NO: 38 - protein, 541 aa, synthetic construct
  source 1..541: note = VAMP4-OVA
MPPKFKRHLNDDDVTGSVKSERRNLLEDDSDEEEDFFLRGPSGPRFGPRNDKIKHVQNQVDEVIDVMQENITKVIERGERLDELQDKSESLSDNATAFSNRSKQLRRQMWWRGCKIKAIMALVAAILLLVIIILIVMKYRTGGGGSGGGGSGGGGSGSIGAASMEFCFDVFKELKVHHANENIFYCPIAIMSALAMVYLGAKDSTRTQINKVVRFDKLPGFGDSIEAQCGTSVNVHSSLRDILNQITKPNDVYSFSLASRLYAEERYPILPEYLQCVKELYRGGLEPINFQTAADQARELINSWVESQTNGIIRNVLQPSSVDSQTAMVLVNAIVFKGLWEKTFKDEDTQAMPFRVTEQESKPVQMMYQIGLFRVASMASEKMKILELPFASGTMSMLVLLPDEVSGLEQLESIINFEKLTEWTSSNVMEERKIKVYLPRMKMEEKYNLTSVLMAMGITDVFSSSANLSGISSAESLKISQAVHAAHAEINEAGREVVGSAEAGVDAASVSEEFRADHPFLFCIKHIATNAVLFFGRCVSP

SEQ ID NO: 39 - protein, 500 aa, synthetic construct
  source 1..500: note = VAMP8-OVA
MEEASEGGGNDRVRNLQSEVEGVKNIMTQNVERILARGENLEHLRNKTEDLEATSEHFKTTSQKVARKFWWKNVKMIVLICVIVFIIILFIVLFATGAFSGGGGSGGGGSGGGGSGSIGAASMEFCFDVFKELKVHHANENIFYCPIAIMSALAMVYLGAKDSTRTQINKVVRFDKLPGFGDSIEAQCGTSVNVHSSLRDILNQITKPNDVYSFSLASRLYAEERYPILPEYLQCVKELYRGGLEPINFQTAADQARELINSWVESQTNGIIRNVLQPSSVDSQTAMVLVNAIVFKGLWEKTFKDEDTQAMPFRVTEQESKPVQMMYQIGLFRVASMASEKMKILELPFASGTMSMLVLLPDEVSGLEQLESIINFEKLTEWTSSNVMEERKIKVYLPRMKMEEKYNLTSVLMAMGITDVFSSSANLSGISSAESLKISQAVHAAHAEINEAGREVVGSAEAGVDAASVSEEFRADHPFLFCIKHIATNAVLFFGRCVSP

SEQ ID NO: 40 - protein, 632 aa, synthetic construct
  source 1..632: note = VTI1B-OVA
MASSAASSEHFEKLHEIFRGLHEDLQGVPERLLGTAGTEEKKKLIRDFDEKQQEANETLAEMEEELRYAPLSFRNPMMSKLRNYRKDLAKLHREVRSTPLTATPGGRGDMKYGIYAVENEHMNRLQSQRAMLLQGTESLNRATQSIERSHRIATETDQIGSEIIEELGEQRDQLERTKSRLVNTSENLSKSRKILRSMSRKVTTNKLLLSIIILLELAILGGLVYYKFFRSHGGGGSGGGGSGGGGSGSIGAASMEFCFDVFKELKVHHANENIFYCPIAIMSALAMVYLGAKDSTRTQINKVVRFDKLPGFGDSIEAQCGTSVNVHSSLRDILNQITKPNDVYSFSLASRLYAEERYPILPEYLQCVKELYRGGLEPINFQTAADQARELINSWVESQTNGIIRNVLQPSSVDSQTAMVLVNAIVFKGLWEKTFKDEDTQAMPFRVTEQESKPVQMMYQIGLFRVASMASEKMKILELPFASGTMSMLVLLPDEVSGLEQLESIINFEKLTEWTSSNVMEERKIKVYLPRMKMEEKYNLTSVLMAMGITDVFSSSANLSGISSAESLKISQAVHAAHAEINEAGREVVGSAEAGVDAASVSEEFRADHPFLFCIKHIATNAVLFFGRCVSP

SEQ ID NO: 41 - protein, 650 aa, synthetic construct
  source 1..650: note = GOSR1-OVA
MAAGTSSYWEDLRKQARQLENELDLKLVSFSKLCTSYSHSSTRDGRRDRYSSDTTPLLNGSSQDRMFETMAIEIEQLLARLTGVNDKMAEYTNSAGVPSLNAALMHTLQRHRDILQDYTHEFHKTKANFMAIRERENLMGSVRKDIESYKSGSGVNNRRTELFLKEHDHLRNSDRLIEETISIAMATKENMTSQRGMLKSIHSKMNTLANRFPAVNSLIQRINLRKRRDSLILGGVIGICTILLLLYAFHGGGGSGGGGSGGGGSGSIGAASMEFCFDVFKELKVHHANENIFYCPIAIMSALAMVYLGAKDSTRTQINKVVRFDKLPGFGDSIEAQCGTSVNVHSSLRDILNQITKPNDVYSFSLASRLYAEERYPILPEYLQCVKELYRGGLEPINFQTAADQARELINSWVESQTNGIIRNVLQPSSVDSQTAMVLVNAIVFKGLWEKTFKDEDTQAMPFRVTEQESKPVQMMYQIGLFRVASMASEKMKILELPFASGTMSMLVLLPDEVSGLEQLESIINFEKLTEWTSSNVMEERKIKVYLPRMKMEEKYNLTSVLMAMGITDVFSSSANLSGISSAESLKISQAVHAAHAEINEAGREVVGSAEAGVDAASVSEEFRADHPFLFCIKHIATNAVLFFGRCVSP

SEQ ID NO: 42 - protein, 518 aa, synthetic construct
  source 1..518: note = BET1-OVA
MRRAGLGEGVPPGNYGNYGYANSGYSACEEENERLTESLRSKVTAIKSLSIEIGHEVKTQNKLLAEMDSQFDSTTGFLGKTMGKLKILSRGSQTKLLCYMMLFSLFVFFIIYWIIKLRGGGGSGGGGSGGGGSGSIGAASMEFCFDVFKELKVHHANENIFYCPIAIMSALAMVYLGAKDSTRTQINKVVRFDKLPGFGDSIEAQCGTSVNVHSSLRDILNQITKPNDVYSFSLASRLYAEERYPILPEYLQCVKELYRGGLEPINFQTAADQARELINSWVESQTNGIIRNVLQPSSVDSQTAMVLVNAIVFKGLWEKTFKDEDTQAMPFRVTEQESKPVQMMYQIGLFRVASMASEKMKILELPFASGTMSMLVLLPDEVSGLEQLESIINFEKLTEWTSSNVMEERKIKVYLPRMKMEEKYNLTSVLMAMGITDVFSSSANLSGISSAESLKISQAVHAAHAEINEAGREVVGSAEAGVDAASVSEEFRADHPFLFCIKHIATNAVLFFGRCVSP

SEQ ID NO: 43 - protein, 690 aa, synthetic construct
  source 1..690: note = BET1L-OVA
MAFCAILLVPSLCRMPSLPTSPWAFPVHWAGFMFKPLDWQGNDFFPPQDEVLAPCLGIKTPLKHEPCASLPFSVLFQSSASQSLLGTMGSLSPHLCGHTMCPVNPELPLSFQADHRSAQPDACSPLCHPSSLLPSFHTASLPFSIHAHHSPLPCDLDPPLYLAETVSLLEEWGPPSSCPMQCKLTSHPARLTHLPPCLWGFAVALKPSWAGLAPSLLPPPRMSLCRPLSFLRHQCPWLPWQAHQGLVPWSPSMVAAACIVSPSGHCRCQPFIPHVFLGHGGLTSVSGECGGGGGSGGGGSGGGGSGSIGAASMEFCFDVFKELKVHHANENIFYCPIAIMSALAMVYLGAKDSTRTQINKVVRFDKLPGFGDSIEAQCGTSVNVHSSLRDILNQITKPNDVYSFSLASRLYAEERYPILPEYLQCVKELYRGGLEPINFQTAADQARELINSWVESQTNGIIRNVLQPSSVDSQTAMVLVNAIVFKGLWEKTFKDEDTQAMPFRVTEQESKPVQMMYQIGLFRVASMASEKMKILELPFASGTMSMLVLLPDEVSGLEQLESIINFEKLTEWTSSNVMEERKIKVYLPRMKMEEKYNLTSVLMAMGITDVFSSSANLSGISSAESLKISQAVHAAHAEINEAGREVVGSAEAGVDAASVSEEFRADHPFLFCIKHIATNAVLFFGRCVSP

SEQ ID NO: 44 - protein, 615 aa, synthetic construct
  source 1..615: note = SEC22B-OVA
MVLLTMIARVADGLPLAASMQEDEQSGRDLQQYQSQAKQLFRKLNEQSPTRCTLEAGAMTFHYIIEQGVCYLVLCEAAFPKKLAFAYLEDLHSEFDEQHGKKVPTVSRPYSFIEFDTFIQKTKKLYIDSRARRNLGSINTELQDVQRIMVANIEEVLQRGEALSALDSKANNLSSLSKKYRQDAKYLNMRSTYAKLAAVAVFFIMLIVYVRFWWLGGGGSGGGGSGGGGSGSIGAASMEFCFDVFKELKVHHANENIFYCPIAIMSALAMVYLGAKDSTRTQINKVVRFDKLPGFGDSIEAQCGTSVNVHSSLRDILNQITKPNDVYSFSLASRLYAEERYPILPEYLQCVKELYRGGLEPINFQTAADQARELINSWVESQTNGIIRNVLQPSSVDSQTAMVLVNAIVFKGLWEKTFKDEDTQAMPFRVTEQESKPVQMMYQIGLFRVASMASEKMKILELPFASGTMSMLVLLPDEVSGLEQLESIINFEKLTEWTSSNVMEERKIKVYLPRMKMEEKYNLTSVLMAMGITDVFSSSANLSGISSAESLKISQAVHAAHAEINEAGREVVGSAEAGVDAASVSEEFRADHPFLFCIKHIATNAVLFFGRCVSP

SEQ ID NO: 45 - protein, 659 aa, synthetic construct
  source 1..659: note = USE1-OVA
MAASRLELNLVRLLSRCEAMAAEKRDPDEWRLEKYVGALEDMLQALKVHASKPASEVINEYSWKVDFLKGMLQAEKLTSSSEKALANQFLAPGRVPTTARERVPATKTVHLQSRARYTSEMRSELLGTDSAEPEMDVRKRTGVAGSQPVSEKQLAAELDLVLQRHQNLQEKLAEEMLGLARSLKTNTLAAQSVIKKDNQTLSHSLKMADQNLEKLKTESERLEQHTQKSVNWLLWAMLIIVCFIFISMILFIRIMPKLKGGGGSGGGGSGGGGSGSIGAASMEFCFDVFKELKVHHANENIFYCPIAIMSALAMVYLGAKDSTRTQINKVVRFDKLPGFGDSIEAQCGTSVNVHSSLRDILNQITKPNDVYSFSLASRLYAEERYPILPEYLQCVKELYRGGLEPINFQTAADQARELINSWVESQTNGIIRNVLQPSSVDSQTAMVLVNAIVFKGLWEKTFKDEDTQAMPFRVTEQESKPVQMMYQIGLFRVASMASEKMKILELPFASGTMSMLVLLPDEVSGLEQLESIINFEKLTEWTSSNVMEERKIKVYLPRMKMEEKYNLTSVLMAMGITDVFSSSANLSGISSAESLKISQAVHAAHAEINEAGREVVGSAEAGVDAASVSEEFRADHPFLFCIKHIATNAVLFFGRCVSP

SEQ ID NO: 46 - protein, 626 aa, synthetic construct
  source 1..626: note = VAMP7-pc-OVA
MAILFAVVARGTTILAKHAWCGGNFLEVTEQILAKIPSENNKLTYSHGNYLFHYICQDRIVYLCITDDDFERSRAFNFLNEIKKRFQTTYGSRAQTALPYAMNSEFSSVLAAQLKHHSENKGLDKVMETQAQVDELKGIMVRNIDLVAQRGERLELLIDKTENLVDSSVTFKTTSRNLARAMCMKNLKLTIIIIIVSIVFIYIIVSPLCGGFTWPSCVKKSGGGGSGGGGSGGGGSRRARRGSIGAASMEFCFDVFKELKVHHANENIFYCPIAIMSALAMVYLGAKDSTRTQINKVVRFDKLPGFGDSIEAQCGTSVNVHSSLRDILNQITKPNDVYSFSLASRLYAEERYPILPEYLQCVKELYRGGLEPINFQTAADQARELINSWVESQTNGIIRNVLQPSSVDSQTAMVLVNAIVFKGLWEKTFKDEDTQAMPFRVTEQESKPVQMMYQIGLFRVASMASEKMKILELPFASGTMSMLVLLPDEVSGLEQLESIINFEKLTEWTSSNVMEERKIKVYLPRMKMEEKYNLTSVLMAMGITDVFSSSANLSGISSAESLKISQAVHAAHAEINEAGREVVGSAEAGVDAASVSEEFRADHPFLFCIKHIATNAVLFFGRCVSP

SEQ ID NO: 47 - protein, 802 aa, synthetic construct
  source 1..802: note = LAMP[OVA]
MAAPGSARRPLLLLLLLLLLGLMHCASAAMFMVKNGNGTACIMANFSAAFSVNYDTKSGPKNMTFDLPSDATVVLNRSSCGKENTSDPSLVIAFGRGHTLTLNFTRNATRYSVQLMSFVYNLSDTHLFPNASSKEIKTVESITDIRADIDKKYRCVSGTQVHMNNVTVTLHDATIQAYLSNSSFSRGETRCEQDRPSPTTAPPAPPSPSPSPVPKSPSVDKYNVSGTNGTCLLASMGLQLNLTYERKDNTTVTRLLNINPNKTSASGSCGAHLVTLELHSEGTTVLLFQFGMNASSSRFFLQGIQLNTILPDARDPAFKAANGSLRALQATVGNSYKCNAEEHVRVTKAFSVNIFKVWVQAFKVEGGQFGSVEECLLDENSMGSIGAASMEFCFDVFKELKVHHANENIFYCPIAIMSALAMVYLGAKDSTRTQINKVVRFDKLPGFGDSIEAQCGTSVNVHSSLRDILNQITKPNDVYSFSLASRLYAEERYPILPEYLQCVKELYRGGLEPINFQTAADQARELINSWVESQTNGIIRNVLQPSSVDSQTAMVLVNAIVFKGLWEKTFKDEDTQAMPFRVTEQESKPVQMMYQIGLFRVASMASEKMKILELPFASGTMSMLVLLPDEVSGLEQLESIINFEKLTEWTSSNVMEERKIKVYLPRMKMEEKYNLTSVLMAMGITDVFSSSANLSGISSAESLKISQAVHAAHAEINEAGREVVGSAEAGVDAASVSEEFRADHPFLFCIKHIATNAVLFFGRCVSPLIPIAVGGALAGLVLIVLIAYLVGRKRSHAGYQTI

SEQ ID NO: 48 - DNA, 1866 bp, synthetic construct
  source 1..1866: mol_type = other DNA; note = VAMP7-OVA
atggccatcctgttcgccgtggtggctagaggcacaaccattctggccaagcacgcttggtgcggcggcaactttctggaagtgaccgagcagatcctggccaagattcccagcgagaacaacaagctgacctacagccacggcaactacctgttccactacatctgccaggaccggatcgtgtacctgtgcatcaccgacgacgacttcgagcggagcagagccttcaacttcctgaacgagatcaagaagcggttccagaccacctacggcagcagagcacaaacagccctgccttacgccatgaacagcgagttcagctctgtgctggccgctcagctgaagcaccactccgagaacaaaggcctggacaaagtgatggaaacacaggcccaggtggacgagctgaagggcatcatggtccgaaacatcgacctggtggcccagagaggcgagagactggaactgctgatcgacaagaccgagaacctggtggacagcagcgtgaccttcaagaccaccagcagaaacctggccagagccatgtgcatgaagaacctgaagctgacgatcatcatcattatcgtgtccatcgtgttcatctacatcatcgtgtccccactgtgtggcggcttcacctggcctagctgtgtgaagaaatctggcggcggaggatctggcggaggtggaagcggaggcggaggaagtggatctattggagccgccagcatggaattttgcttcgacgtgttcaaagaactgaaggtgcaccacgccaacgagaacatcttctactgccctatcgccatcatgagcgccctggctatggtgtatctgggcgccaaggacagcacccggacacagatcaacaaggtcgtcagattcgacaagctgcccggcttcggcgattctatcgaagcccagtgtggcaccagcgtgaacgtgcacagcagcctgagagacatcctgaatcagatcaccaagcctaacgacgtgtactccttcagcctggccagcagactgtacgccgaggaaagataccccatcctgcctgagtacctgcagtgcgtgaaagagctgtacagaggcggcctggaacctatcaacttccagacagccgccgaccaggccagagagctgatcaattcttgggtcgagagccagaccaacggcatcatcagaaacgtgctgcagcccagctccgtggattctcagacagccatggtgctggtcaacgccattgtgtttaaaggcctgtgggagaaaaccttcaaggacgaggacacccaggccatgcctttcagagtgacagagcaagagtccaagcctgtgcagatgatgtaccagatcggcctgtttagagtggcctccatggcctccgagaagatgaagatcctcgagctgcctttcgccagcggcaccatgtctatgctggtgctgctgcctgatgaggtgtccggactggaacagctcgagagcatcatcaacttcgagaagctgaccgagtggaccagcagcaacgtgatggaagaacggaagatcaaggtgtacctgcctcggatgaagatggaagagaagtacaacctgaccagcgtgctgatggctatgggcatcacagacgtgttctccagcagcgccaatctgagcggcatcagctctgccgagagcctgaagatttctcaggccgtgcatgctgcccacgccgagattaacgaagccggcagagaagttgtgggatctgccgaagcaggcgtggacgctgcttctgtgtctgaggaattccgggccgaccatccttttctgttctgcatcaagcacattgccaccaacgccgtgctgttctttggcagatgcgtgtccccttga

SEQ ID NO: 49 - DNA, 1974 bp, synthetic construct
  source 1..1974: mol_type = other DNA; note = GOSR2-OVA
atggatcctctgttccagcagacccacaaacaggtgcacgagatccagagctgcatgggcagactggaaaccgccgataagcagagcgtgcacatcgtggaaaatgagatccaggccagcatcgaccagatcttcagcaggctggaacggctggaaatcctgagcagcaaagagcctcctaacaagcggcagaacgcccggctgagagtggaccagctgaagtacgatgtccagcacctccagacagccctgcggaactttcagcacagaaggcacgccagagagcagcaagaacggcagagagaggaactgctgagccggaccttcaccaccaacgacagcgacaccaccattcctatggacgagagcctgcagttcaacagcagcctgcagaaagtgcacaacggcatggacgacctgatcctggacggccacaatatcctggatggcctgagaacccagcggctgacactgaagggcacccagaagaagatcctggatatcgccaacatgctgggcctgagcaacaccgtgatgcggctgattgagaagcgggccttccaggacaagtacttcatgatcgagacacggtcccaccacgtggcccagaatggacctgaactgctgtccagcagagatcctcctgccagcgcctctagatctgccggcatcatcggcatgagccaccatcctgacctgcagatccctttcgagctgagactgggcttcgagctgtggttctatcagctgctggccgtgatcagcgaccaaggcggcggaggatctggcggaggtggaagcggaggcggaggaagtggatctattggagccgccagcatggaattttgcttcgacgtgttcaaagaactgaaggtgcaccacgccaacgagaacatcttctactgccctatcgccatcatgagcgccctggctatggtgtatctgggcgccaaggacagcacccggacacagatcaacaaggtcgtcagattcgacaagctgcccggcttcggcgattctatcgaagcccagtgtggcaccagcgtgaacgtgcacagcagcctgagagacatcctgaatcagatcaccaagcctaacgacgtgtactccttcagcctggccagcagactgtacgccgaggaaagataccccatcctgcctgagtacctgcagtgcgtgaaagagctgtacagaggcggcctggaacctatcaacttccagacagccgccgaccaggccagagagctgatcaattcttgggtcgagagccagaccaacggcatcatcagaaacgtgctgcagcccagctccgtggattctcagacagccatggtgctggtcaacgccattgtgtttaaaggcctgtgggagaaaaccttcaaggacgaggacacccaggccatgcctttcagagtgacagagcaagagtccaagcctgtgcagatgatgtaccagatcggcctgtttagagtggcctccatggcctccgagaagatgaagatcctcgagctgcctttcgccagcggcaccatgtctatgctggtgctgctgcctgatgaggtgtccggactggaacagctcgagagcatcatcaacttcgagaagctgaccgagtggaccagcagcaacgtgatggaagaacggaagatcaaggtgtacctgcctcggatgaagatggaagagaagtacaacctgaccagcgtgctgatggctatgggcatcacagacgtgttctccagcagcgccaatctgagcggcatcagctctgccgagagcctgaagatttctcaggccgtgcatgctgcccacgccgagattaacgaagccggcagagaagttgtgggatctgccgaagcaggcgtggacgctgcttctgtgtctgaggaattccgggccgaccatccttttctgttctgcatcaagcacattgccaccaacgccgtgctgttctttggcagatgcgtgtccccttga

SEQ ID NO: 50 - DNA, 1950 bp, synthetic construct
  source 1..1950: mol_type = other DNA; note = STX10-OVA
atgagcctggaagatcccttctttgtcgtgcgcggcgaggtgcagaaagccgtgaatactgccagaggcctgtaccagcgttggtgcgagctgctgcaagaatctgccgctgtgggcagagaggaactggactggaccaccaacgagctgagaaacggcctgagatccatcgagtgggacctcgaggacctggaagagacaatcggcatcgtggaagccaatcctggcaagttcaaactgcctgccggcgacctgcaagagcggaaggtgttcgtggaacggatgcgggaagccgtgcaagagatgaaggaccacatggtgtctccaaccgccgtggccttcctggaacggaacaacagagagatcctggccggaaagcctgccgctcagaagtctcctagcgatctgctggatgcctctgccgtgtctgccacaagccggtacattgaggaacagcaggccacacagcagctgatcatggacgagcaggaccagcagctggaaatggtgtctggcagcatccaggtgctgaagcacatgagcggaagagtgggcgaagaactggatgagcagggcatcatgctggacgccttcgctcaagagatggatcacacccagagccggatggacggcgtgctgagaaagctggccaaagtgtcccacatgaccagcgaccgtagacagtggtgcgccattgctgtgcttgtgggagtgctgctgctggtgctgatcctgctgtttagccttggcggcggaggatctggcggaggtggaagcggaggcggaggaagtggatctattggagccgccagcatggaattttgcttcgacgtgttcaaagaactgaaggtgcaccacgccaacgagaacatcttctactgccctatcgccatcatgagcgccctggctatggtgtatctgggcgccaaggacagcacccggacacagatcaacaaggtcgtcagattcgacaagctgcccggcttcggcgattctatcgaagcccagtgtggcaccagcgtgaacgtgcacagcagcctgagagacatcctgaatcagatcaccaagcctaacgacgtgtactccttcagcctggccagcagactgtacgccgaggaaagataccccatcctgcctgagtacctgcagtgcgtgaaagagctgtacagaggcggcctggaacctatcaacttccagacagccgccgaccaggccagagagctgatcaattcttgggtcgagagccagaccaacggcatcatcagaaacgtgctgcagcccagctccgtggattctcagacagccatggtgctggtcaacgccattgtgtttaaaggcctgtgggagaaaaccttcaaggacgaggacacccaggccatgcctttcagagtgacagagcaagagtccaagcctgtgcagatgatgtaccagatcggcctgtttagagtggcctccatggcctccgagaagatgaagatcctcgagctgcctttcgccagcggcaccatgtctatgctggtgctgctgcctgatgaggtgtccggactggaacagctcgagagcatcatcaacttcgagaagctgaccgagtggaccagcagcaacgtgatggaagaacggaagatcaaggtgtacctgcctcggatgaagatggaagagaagtacaacctgaccagcgtgctgatggctatgggcatcacagacgtgttctccagcagcgccaatctgagcggcatcagctctgccgagagcctgaagatttctcaggccgtgcatgctgcccacgccgagattaacgaagccggcagagaagttgtgggatctgccgaagcaggcgtggacgctgcttctgtgtctgaggaattccgggccgaccatccttttctgttctgcatcaagcacattgccaccaacgccgtgctgttctttggcagatgcgtgtccccttga

SEQ ID NO: 51 - DNA, 2208 bp, synthetic construct
  source 1..2208: mol_type = other DNA; note = STX18-OVA
atggccgtggatatcaccctgctgtttcgggccagcgtgaaaacagtgaaaacccggaacaaggccctgggcgttgcagttggaggcggagttgatggcagcagggatgagctgttcagaagaagccccagacctaagggcgacttcagcagcagagcccgggaagtgatcagccacatcggcaagctgagagacttcctgctggaacaccggaaggactacatcaacgcctacagccacaccatgagcgagtacggcagaatgaccgacaccgagagggaccagatcgaccaggatgcccagatcttcatgcggacctgtagcgaggccatccagcagctgagaacagaggcccacaaagagatccacagccagcaagtgaaagaacacagaaccgccgtgctggacttcatcgaggactacctgaagagagtgtgcaagctgtactccgagcagcgggccatcagagtgaaaagagtggtggacaagaagcggctgagcaagctggaacccgagcctaacaccaagaccagagagagcaccagctccgagaaagtgtctcagagccccagcaaggacagcgaggaaaatcctgccaccgaggaacggcccgagaagattctggctgagacacagcctgaactcggcacctggggagatggcaagggcgaagatgaactgagccccgaagagattcagatgttcgagcaagagaaccagcggctgatcggcgagatgaacagcctgtttgacgaagtgcggcagatcgagggccgcgtggtggaaatctctcggctgcaagagatcttcaccgagaaggtcctgcagcaagaggccgagatcgacagcatccatcagctggttgtgggcgccaccgagaacatcaaagagggcaacgaggacatcagagaggccatcaagaacaacgccggcttcagagtgtggatcctgttcttcctggtcatgtgcagcttcagcctgctgttcctggattggtacgactctggcggcggaggatctggcggaggtggaagcggaggcggaggaagtggatctattggagccgccagcatggaattttgcttcgacgtgttcaaagaactgaaggtgcaccacgccaacgagaacatcttctactgccctatcgccatcatgagcgccctggctatggtgtatctgggcgccaaggacagcacccggacacagatcaacaaggtcgtcagattcgacaagctgcccggcttcggcgattctatcgaagcccagtgtggcaccagcgtgaacgtgcacagcagcctgagagacatcctgaatcagatcaccaagcctaacgacgtgtactccttcagcctggccagcagactgtacgccgaggaaagataccccatcctgcctgagtacctgcagtgcgtgaaagagctgtacagaggcggcctggaacctatcaacttccagacagccgccgaccaggccagagagctgatcaattcttgggtcgagagccagaccaacggcatcatcagaaacgtgctgcagcccagctccgtggattctcagacagccatggtgctggtcaacgccattgtgtttaaaggcctgtgggagaaaaccttcaaggacgaggacacccaggccatgcctttcagagtgacagagcaagagtccaagcctgtgcagatgatgtaccagatcggcctgtttagagtggcctccatggcctccgagaagatgaagatcctcgagctgcctttcgccagcggcaccatgtctatgctggtgctgctgcctgatgaggtgtccggactggaacagctcgagagcatcatcaacttcgagaagctgaccgagtggaccagcagcaacgtgatggaagaacggaagatcaaggtgtacctgcctcggatgaagatggaagagaagtacaacctgaccagcgtgctgatggctatgggcatcacagacgtgttctccagcagcgccaatctgagcggcatcagctctgccgagagcctgaagatttctcaggccgtgcatgctgcccacgccgagattaacgaagccggcagagaagttgtgggatctgccgaagcaggcgtggacgctgcttctgtgtctgaggaattccgggccgaccatccttttctgttctgcatcaagcacattgccaccaacgccgtgctgttctttggcagatgcgtgtccccttga

SEQ ID NO: 52 - DNA, 2016 bp, synthetic construct
  source 1..2016: mol_type = other DNA; note = BNIP1-OVA
atggctgctcctcaggatgtgcacgtgcggatctgcaatcaagagatcgtgaagttcgacctggaagtgaaggccctgatccaggacatcagagactgtagcggacctctgagcgccctgaccgagctgaacaccaaagtgaaagagaagttccagcagctgcggcaccggatccagcctgtgctgtatcagagagccttcatctggaccgccagcaccttctttttcaaactgacctacagcctgaccgacttcagcagcacccagcacgacttcaacagccctaccacacctgtgaccttcagcgatctggaacagctggccaaagagcaggacaaagagagcgagaaacagctgctgctgcaagaggtggaaaaccacaaaaagcagatgctgagcaaccaggcctcctggcggaaggccaatctgacatgcaagatcgccatcgacaacctggaaaaggccgagctgctccaaggcggcgatctgctgagacagagaaagaccaccaaagagtctctggcccagaccagctccaccatcaccgaatctctgatgggcatcagcagaatgatggcccagcaggtccagcagagcgaggaagccatgcagagcctggtcaccagcagcagaacaatcctggacgccaacgaggaattcaagagcatgagcggcaccatccagctgggcagaaagctgatcaccaagtacaacagaagagagctgaccgacaagctgctgatcttcctggctctggccctgtttctggccaccgtgctgtacatcgtgaagaagcggctgttcccattccttggcggcggaggatctggcggaggtggaagcggaggcggaggaagtggatctattggagccgccagcatggaattttgcttcgacgtgttcaaagaactgaaggtgcaccacgccaacgagaacatcttctactgccctatcgccatcatgagcgccctggctatggtgtatctgggcgccaaggacagcacccggacacagatcaacaaggtcgtcagattcgacaagctgcccggcttcggcgattctatcgaagcccagtgtggcaccagcgtgaacgtgcacagcagcctgagagacatcctgaatcagatcaccaagcctaacgacgtgtactccttcagcctggccagcagactgtacgccgaggaaagataccccatcctgcctgagtacctgcagtgcgtgaaagagctgtacagaggcggcctggaacctatcaacttccagacagccgccgaccaggccagagagctgatcaattcttgggtcgagagccagaccaacggcatcatcagaaacgtgctgcagcccagctccgtggattctcagacagccatggtgctggtcaacgccattgtgtttaaaggcctgtgggagaaaaccttcaaggacgaggacacccaggccatgcctttcagagtgacagagcaagagtccaagcctgtgcagatgatgtaccagatcggcctgtttagagtggcctccatggcctccgagaagatgaagatcctcgagctgcctttcgccagcggcaccatgtctatgctggtgctgctgcctgatgaggtgtccggactggaacagctcgagagcatcatcaacttcgagaagctgaccgagtggaccagcagcaacgtgatggaagaacggaagatcaaggtgtacctgcctcggatgaagatggaagagaagtacaacctgaccagcgtgctgatggctatgggcatcacagacgtgttctccagcagcgccaatctgagcggcatcagctctgccgagagcctgaagatttctcaggccgtgcatgctgcccacgccgagattaacgaagccggcagagaagttgtgggatctgccgaagcaggcgtggacgctgcttctgtgtctgaggaattccgggccgaccatccttttctgttctgcatcaagcacattgccaccaacgccgtgctgttctttggcagatgcgtgtccccttga

SEQ ID NO: 53 - DNA, 1986 bp, synthetic construct
  source 1..1986: mol_type = other DNA; note = STX7-OVA
atgagctacacacctggcgttggcggagatcctgctcagctggcccagagaatcagcagcaacatccagaaaatcacccagtgcagcgtggaaatccagcggaccctgaatcagctgggcacccctcaggatagccctgagctgagacagcagctgcagcagaagcagcagtacaccaaccagctggccaaagagacagacaagtacatcaaagagttcggcagcctgcctaccacacctagcgagcagagacagcggaagatccagaaagacagactggtggccgagttcaccaccagcctgaccaacttccagaaggtgcagaggcaggccgctgagcgcgagaaagaatttgtggccagagtgcgggccagcagcagagtgtcaggatcctttccagaggacagctccaaagagcggaacctggtttcctgggagagccagacacagcctcaggtgcaggtccaggacgaggaaatcaccgaggacgacctgagactgatccacgagagagagtccagcatccggcagctggaagccgacatcatggacatcaacgagatcttcaaggacctgggcatgatgattcacgagcagggcgacgtgatcgacagcatcgaggccaacgtggaaaacgccgaagtgcatgtgcagcaggccaaccagcagctgtctagagccgccgactaccagcgcaagagcagaaagaccctgtgcatcatcatcctgatcctggtcatcggcgtggccatcatctccctgatcatctggggcctgaaccatggcggcggaggatctggcggaggtggaagcggaggcggaggaagtggatctattggagccgccagcatggaattttgcttcgacgtgttcaaagaactgaaggtgcaccacgccaacgagaacatcttctactgccctatcgccatcatgagcgccctggctatggtgtatctgggcgccaaggacagcacccggacacagatcaacaaggtcgtcagattcgacaagctgcccggcttcggcgattctatcgaagcccagtgtggcaccagcgtgaacgtgcacagcagcctgagagacatcctgaatcagatcaccaagcctaacgacgtgtactccttcagcctggccagcagactgtacgccgaggaaagataccccatcctgcctgagtacctgcagtgcgtgaaagagctgtacagaggcggcctggaacctatcaacttccagacagccgccgaccaggccagagagctgatcaattcttgggtcgagagccagaccaacggcatcatcagaaacgtgctgcagcccagctccgtggattctcagacagccatggtgctggtcaacgccattgtgtttaaaggcctgtgggagaaaaccttcaaggacgaggacacccaggccatgcctttcagagtgacagagcaagagtccaagcctgtgcagatgatgtaccagatcggcctgtttagagtggcctccatggcctccgagaagatgaagatcctcgagctgcctttcgccagcggcaccatgtctatgctggtgctgctgcctgatgaggtgtccggactggaacagctcgagagcatcatcaacttcgagaagctgaccgagtggaccagcagcaacgtgatggaagaacggaagatcaaggtgtacctgcctcggatgaagatggaagagaagtacaacctgaccagcgtgctgatggctatgggcatcacagacgtgttctccagcagcgccaatctgagcggcatcagctctgccgagagcctgaagatttctcaggccgtgcatgctgcccacgccgagattaacgaagccggcagagaagttgtgggatctgccgaagcaggcgtggacgctgcttctgtgtctgaggaattccgggccgaccatccttttctgttctgcatcaagcacattgccaccaacgccgtgctgttctttggcagatgcgtgtccccttga

SEQ ID NO: 54 - DNA, 1875 bp, synthetic construct
  source 1..1875: mol_type = other DNA; note = VTI1A-OVA
atgagcagcgacttcgagggctacgagcaggattttgccgtgctgaccgccgagatcaccagcaagattgccagagtgcccagactgcctcctgacgagaagaaacagatggtggccaacgtggaaaagcagctggaagaggccaaagaactgctggaacagatggacctggaagtgcgcgagatccctccacagagcagaggcatgtacagcaaccggatgcggagctacaagcaagagatgggcaagctggaaaccgacttcaagcggagcagaatcgcctacagcgacgaagtgcggaatgagctgctgggcgacgatggcaacagcagcgagaaccagctgatcaagctgcgggaagagagagcccatctgctggacaacaccgagcggctggaaagaagcagcagaaggctggaagccggctatcagatcgccgtggaaactgagcagatcggccaagagatgctggaaaacctgagccacgacagagagaagatccagcgggccagagagcggctgagagagacagacgccaatctgggcaagagcagcaggattctgaccggcatgctgcggcggatcatccagaataggatcctgctggtcatcctgggcatcatcgtggtcatcaccatcctgatggccattaccttcagcgtgcggcggcatggcggcggaggatctggcggaggtggaagcggaggcggaggaagtggatctattggagccgccagcatggaattttgcttcgacgtgttcaaagaactgaaggtgcaccacgccaacgagaacatcttctactgccctatcgccatcatgagcgccctggctatggtgtatctgggcgccaaggacagcacccggacacagatcaacaaggtcgtcagattcgacaagctgcccggcttcggcgattctatcgaagcccagtgtggcaccagcgtgaacgtgcacagcagcctgagagacatcctgaatcagatcaccaagcctaacgacgtgtactccttcagcctggccagcagactgtacgccgaggaaagataccccatcctgcctgagtacctgcagtgcgtgaaagagctgtacagaggcggcctggaacctatcaacttccagacagccgccgaccaggccagagagctgatcaattcttgggtcgagagccagaccaacggcatcatcagaaacgtgctgcagcccagctccgtggattctcagacagccatggtgctggtcaacgccattgtgtttaaaggcctgtgggagaaaaccttcaaggacgaggacacccaggccatgcctttcagagtgacagagcaagagtccaagcctgtgcagatgatgtaccagatcggcctgtttagagtggcctccatggcctccgagaagatgaagatcctcgagctgcctttcgccagcggcaccatgtctatgctggtgctgctgcctgatgaggtgtccggactggaacagctcgagagcatcatcaacttcgagaagctgaccgagtggaccagcagcaacgtgatggaagaacggaagatcaaggtgtacctgcctcggatgaagatggaagagaagtacaacctgaccagcgtgctgatggctatgggcatcacagacgtgttctccagcagcgccaatctgagcggcatcagctctgccgagagcctgaagatttctcaggccgtgcatgctgcccacgccgagattaacgaagccggcagagaagttgtgggatctgccgaagcaggcgtggacgctgcttctgtgtctgaggaattccgggccgaccatccttttctgttctgcatcaagcacattgccaccaacgccgtgctgttctttggcagatgcgtgtccccttga

SEQ ID NO: 55 - DNA, 2178 bp, synthetic construct
  source 1..2178: mol_type = other DNA; note = STX16-OVA
atggccaccagaaggctgacagacgctttcctgctgctgcggaacaacagcatccagaacagacagctgctggccgaacaggtgtccagccacatcacatctagccctctgcacagcagatctatcgccgccgagctggatgagctggccgatgatagaatggccctggtgtccggcatctctctggatcctgaagccgccatcggcgtgaccaaacggcctcctcctaaatgggttgacggcgtggacgagatccagtacgacgtgggcagaatcaagcagaagatgaaggaactggccagcctgcacgacaagcacctgaacagacccacactggacgacagcagcgaggaagaacacgccatcgagatcaccacacaagagatcacccagctgttccaccggtgccagagagctgttcaggccctgccttctagagccagagcctgctctgagcaagagggcagactgctgggaaacgtggtggcttctctggctcaggctctgcaagagctgagcaccagctttagacacgcccagagcggctacctgaagcggatgaagaaccgggaagagagatcccagcacttcttcgacaccagcgtgcccctgatggacgacggcgacgataataccctgtaccacagaggcttcaccgaggaccagctcgtgctggttgagcagaacaccctgatggtggaagaacgcgagcgcgagatcagacagatcgtgcagagcatcagcgacctgaacgagatcttcagagatctgggcgccatgatcgtggaacagggcaccgtgctggaccggatcgactacaatgtggaacagagctgcatcaagaccgaggacggactgaagcagctgcacaaagccgagcagtaccagaaaaagaatcggaagatgctggtcatcctgatcctgttcgtgatcatcatcgtgctgatcgtggtgctcgtgggcgtgaagtctagaggcggcggaggatctggcggaggtggaagcggaggcggaggaagtggatctattggagccgccagcatggaattttgcttcgacgtgttcaaagaactgaaggtgcaccacgccaacgagaacatcttctactgccctatcgccatcatgagcgccctggctatggtgtatctgggcgccaaggacagcacccggacacagatcaacaaggtcgtcagattcgacaagctgcccggcttcggcgattctatcgaagcccagtgtggcaccagcgtgaacgtgcacagcagcctgagagacatcctgaatcagatcaccaagcctaacgacgtgtactccttcagcctggccagcagactgtacgccgaggaaagataccccatcctgcctgagtacctgcagtgcgtgaaagagctgtacagaggcggcctggaacctatcaacttccagacagccgccgaccaggccagagagctgatcaattcttgggtcgagagccagaccaacggcatcatcagaaacgtgctgcagcccagctccgtggattctcagacagccatggtgctggtcaacgccattgtgtttaaaggcctgtgggagaaaaccttcaaggacgaggacacccaggccatgcctttcagagtgacagagcaagagtccaagcctgtgcagatgatgtaccagatcggcctgtttagagtggcctccatggcctccgagaagatgaagatcctcgagctgcctttcgccagcggcaccatgtctatgctggtgctgctgcctgatgaggtgtccggactggaacagctcgagagcatcatcaacttcgagaagctgaccgagtggaccagcagcaacgtgatggaagaacggaagatcaaggtgtacctgcctcggatgaagatggaagagaagtacaacctgaccagcgtgctgatggctatgggcatcacagacgtgttctccagcagcgccaatctgagcggcatcagctctgccgagagcctgaagatttctcaggccgtgcatgctgcccacgccgagattaacgaagccggcagagaagttgtgggatctgccgaagcaggcgtggacgctgcttctgtgtctgaggaattccgggccgaccatccttttctgttctgcatcaagcacattgccaccaacgccgtgctgttctttggcagatgcgtgtccccttga

SEQ ID NO: 56 - DNA, 2268 bp, synthetic construct
  source 1..2268: mol_type = other DNA; note = STX5-OVA
atgattccccggaagagatacggcagcaagaacaccgatcagggcgtgtacctgggcctgagcaaaacacaggtgctgtctccagccacagccggcagctctagctctgatattgctcccctgcctcctcctgtgacactggttcctccaccacctgacaccatgagctgcagagacagaacccaagagttcctgagcgcctgcaagagcctgcagaccagacagaatggcatccagaccaacaagcccgctctgagagccgtgcggcagagaagcgagtttaccctgatggccaagcggatcggcaaggacctgagcaacaccttcgccaagctggaaaagctgaccatcctggccaagagaaagagcctgttcgacgacaaggccgtggaaatcgaggaactgacctacatcatcaagcaggacatcaacagcctgaacaagcagatcgcccagctgcaggacttcgtcagagccaagggaagccagagcggcagacacctccagacacacagcaacaccatcgtggtgtccctgcagagcaagctggcctccatgagcaacgacttcaagagcgtgctggaagtgcggaccgagaacctgaagcagcagcggtctagaagagagcagttcagcagagcccctgtgtctgctctgcccctggctcctaatcatcttggaggcggagctgtggtgctgggagccgaatctcacgcctctaaggacgtggccatcgacatgatggacagcagaaccagccagcagctgcaactgatcgacgagcaggacagctacatccagagcagagccgacaccatgcagaacatcgagagcacaatcgtggaactgggcagcatctttcagcagctggcccacatggtcaaagagcaagaggaaaccatccagcgcatcgacgagaatgtgctgggcgctcagctggatgtggaagccgctcactctgagatcctgaagtactttcagagcgtgaccagcaaccggtggctgatggtcaagatcttcctgatcctgatcgtgttctttattatcttcgtcgtgttcctggctggcggcggaggatctggcggaggtggaagcggaggcggaggaagtggatctattggagccgccagcatggaattttgcttcgacgtgttcaaagaactgaaggtgcaccacgccaacgagaacatcttctactgccctatcgccatcatgagcgccctggctatggtgtatctgggcgccaaggacagcacccggacacagatcaacaaggtcgtcagattcgacaagctgcccggcttcggcgattctatcgaagcccagtgtggcaccagcgtgaacgtgcacagcagcctgagagacatcctgaatcagatcaccaagcctaacgacgtgtactccttcagcctggccagcagactgtacgccgaggaaagataccccatcctgcctgagtacctgcagtgcgtgaaagagctgtacagaggcggcctggaacctatcaacttccagacagccgccgaccaggccagagagctgatcaattcttgggtcgagagccagaccaacggcatcatcagaaacgtgctgcagcccagctccgtggattctcagacagccatggtgctggtcaacgccattgtgtttaaaggcctgtgggagaaaaccttcaaggacgaggacacccaggccatgcctttcagagtgacagagcaagagtccaagcctgtgcagatgatgtaccagatcggcctgtttagagtggcctccatggcctccgagaagatgaagatcctcgagctgcctttcgccagcggcaccatgtctatgctggtgctgctgcctgatgaggtgtccggactggaacagctcgagagcatcatcaacttcgagaagctgaccgagtggaccagcagcaacgtgatggaagaacggaagatcaaggtgtacctgcctcggatgaagatggaagagaagtacaacctgaccagcgtgctgatggctatgggcatcacagacgtgttctccagcagcgccaatctgagcggcatcagctctgccgagagcctgaagatttctcaggccgtgcatgctgcccacgccgagattaacgaagccggcagagaagttgtgggatctgccgaagcaggcgtggacgctgcttctgtgtctgaggaattccgggccgaccatccttttctgttctgcatcaagcacattgccaccaacgccgtgctgttctttggcagatgcgtgtccccttga

SEQ ID NO: 57 - DNA, 1968 bp, synthetic construct
  source 1..1968: mol_type = other DNA; note = STX6-OVA
atgagcatggaagatccattcttcgtggtcaagggcgaagtgcagaaagccgtgaacacagcccagggcctgttccagagatggacagagctgctgcaggaccctagcaccgccaccagagaggaaatcgactggaccaccaacgagctgcggaacaacctgagatccatcgagtgggacctcgaggacctggacgagacaatcagcatcgtggaagccaatcctcggaagttcaacctggacgccaccgagctgagcatcagaaaggccttcatcaccagcaccagacaggtcgtgcgggacatgaaggaccagatgagcacaagctctgtgcaggctctggccgagcggaagaatagacaggctctgctgggcgatagcggcagccagaattggagcaccggcaccacagataagtacggcagactggatagagagctgcagcgggccaacagccacttcatcgaagaacagcaggcccagcagcagctgatcgtcgagcagcaggatgagcagctggaactggtgtctggctctatcggcgtgctgaagaacatgagccagagaatcggcggcgaactggaagaacaggccgtgatgctggaagatttcagccacgagctggaaagcacccagagcaggctggacaacgtgatgaagaagctggccaaggtttcccacatgaccagcgaccgtagacagtggtgcgccattgccatcctgtttgccgtgctgctggtggtgctgatcctgttcctggtgcttggcggcggaggatctggcggaggtggaagcggaggcggaggaagtggatctattggagccgccagcatggaattttgcttcgacgtgttcaaagaactgaaggtgcaccacgccaacgagaacatcttctactgccctatcgccatcatgagcgccctggctatggtgtatctgggcgccaaggacagcacccggacacagatcaacaaggtcgtcagattcgacaagctgcccggcttcggcgattctatcgaagcccagtgtggcaccagcgtgaacgtgcacagcagcctgagagacatcctgaatcagatcaccaagcctaacgacgtgtactccttcagcctggccagcagactgtacgccgaggaaagataccccatcctgcctgagtacctgcagtgcgtgaaagagctgtacagaggcggcctggaacctatcaacttccagacagccgccgaccaggccagagagctgatcaattcttgggtcgagagccagaccaacggcatcatcagaaacgtgctgcagcccagctccgtggattctcagacagccatggtgctggtcaacgccattgtgtttaaaggcctgtgggagaaaaccttcaaggacgaggacacccaggccatgcctttcagagtgacagagcaagagtccaagcctgtgcagatgatgtaccagatcggcctgtttagagtggcctccatggcctccgagaagatgaagatcctcgagctgcctttcgccagcggcaccatgtctatgctggtgctgctgcctgatgaggtgtccggactggaacagctcgagagcatcatcaacttcgagaagctgaccgagtggaccagcagcaacgtgatggaagaacggaagatcaaggtgtacctgcctcggatgaagatggaagagaagtacaacctgaccagcgtgctgatggctatgggcatcacagacgtgttctccagcagcgccaatctgagcggcatcagctctgccgagagcctgaagatttctcaggccgtgcatgctgcccacgccgagattaacgaagccggcagagaagttgtgggatctgccgaagcaggcgtggacgctgcttctgtgtctgaggaattccgggccgaccatccttttctgttctgcatcaagcacattgccaccaacgccgtgctgttctttggcagatgcgtgtccccttga

SEQ ID NO: 58 - DNA, 1911 bp, synthetic construct
  source 1..1911: mol_type = other DNA; note = STX8-OVA
atggctcccgatccatggttcagcacctacgacagcacctgtcagatcgcccaagagatcgccgagaagatccagcagcggaaccagtacgagcggaagggcgagaaagcccctaagctgaccgtgaccattagagccctgctgcagaacctgaaagagaagatcgccctgctgaaggatctgctgctgagagccgtgtctacccaccagatcacacagctggaaggcgaccgcagacagaacctgctggatgacctggtcaccagagagagactgctgctggcctccttcaagaacgaaggcgccgagcctgacctgatcagatccagcctgatgagcgaggaagccaagagaggcgcccctaatccttggctgttcgaggaacccgaggaaaccagaggcctgggcttcgacgagatcagacagcagcagcaaaagatcatccaagagcaggacgccggcctggatgccctgtctagcatcatcagccggcagaaacagatgggccaagagattggcaacgagctggacgagcagaacgagatcatcgacgacctggccaacctggtggaaaacaccgacgagaagctgcggaacgagactcggagagtgaacatggtggaccggaagtctgccagctgcgggatgatcatggttatcctgttgctgctggtggccatcgtggtggtggctgtgtggcctacaaatggcggcggaggatctggcggaggtggaagcggaggcggaggaagtggatctattggagccgccagcatggaattttgcttcgacgtgttcaaagaactgaaggtgcaccacgccaacgagaacatcttctactgccctatcgccatcatgagcgccctggctatggtgtatctgggcgccaaggacagcacccggacacagatcaacaaggtcgtcagattcgacaagctgcccggcttcggcgattctatcgaagcccagtgtggcaccagcgtgaacgtgcacagcagcctgagagacatcctgaatcagatcaccaagcctaacgacgtgtactccttcagcctggccagcagactgtacgccgaggaaagataccccatcctgcctgagtacctgcagtgcgtgaaagagctgtacagaggcggcctggaacctatcaacttccagacagccgccgaccaggccagagagctgatcaattcttgggtcgagagccagaccaacggcatcatcagaaacgtgctgcagcccagctccgtggattctcagacagccatggtgctggtcaacgccattgtgtttaaaggcctgtgggagaaaaccttcaaggacgaggacacccaggccatgcctttcagagtgacagagcaagagtccaagcctgtgcagatgatgtaccagatcggcctgtttagagtggcctccatggcctccgagaagatgaagatcctcgagctgcctttcgccagcggcaccatgtctatgctggtgctgctgcctgatgaggtgtccggactggaacagctcgagagcatcatcaacttcgagaagctgaccgagtggaccagcagcaacgtgatggaagaacggaagatcaaggtgtacctgcctcggatgaagatggaagagaagtacaacctgaccagcgtgctgatggctatgggcatcacagacgtgttctccagcagcgccaatctgagcggcatcagctctgccgagagcctgaagatttctcaggccgtgcatgctgcccacgccgagattaacgaagccggcagagaagttgtgggatctgccgaagcaggcgtggacgctgcttctgtgtctgaggaattccgggccgaccatccttttctgttctgcatcaagcacattgccaccaacgccgtgctgttctttggcagatgcgtgtccccttga

SEQ ID NO: 59 - DNA, 2031 bp, synthetic construct
  source 1..2031: mol_type = other DNA; note = STX12-OVA
atgagctacggccctctggacatgtacagaaaccccggaccttctggcccacagctgagagacttcagcagcatcatccagacctgcagcggcaacatccagagaatcagccaggccaccgctcagatcaagaacctgatgagccagctgggcaccaagcaggacagcagcaagctgcaagagaacctgcagcagctccagcacagcaccaaccagctggccaaagagacaaacgagctgctgaaagagctgggcagcctgcctctgcctctgagcacatctgaacagcggcagcagcggctgcagaaagaacggctgatgaacgacttcagcgccgctctgaacaacttccaggccgtgcagagaagagtgtccgagaaagagaaagagtctatcgccagagccagagccggcagcagactgtctgccgaggaaagacagcgggaagaacagctggtgtccttcgacagccacgaggaatggaaccagatgcagagccaagaggacgaggtggccatcaccgagcaggacctggaactgatcaaagagagagagacagccatccggcagctggaagccgacatcctggatgtgaaccagatcttcaaggacctggccatgatgatccacgaccagggcgacctgatcgacagcatcgaggccaatgtggaaagcagcgaggtgcacgtggaacgggctacagaacaactgcagagagccgcctactaccagaagaaaagccggaagaaaatgtgcatcctggtgctggtcctgagcgtgatcatcctgatcctgggcctgatcatctggctggtgtacaagaccaaaggcggcggaggatctggcggaggtggaagcggaggcggaggaagtggatctattggagccgccagcatggaattttgcttcgacgtgttcaaagaactgaaggtgcaccacgccaacgagaacatcttctactgccctatcgccatcatgagcgccctggctatggtgtatctgggcgccaaggacagcacccggacacagatcaacaaggtcgtcagattcgacaagctgcccggcttcggcgattctatcgaagcccagtgtggcaccagcgtgaacgtgcacagcagcctgagagacatcctgaatcagatcaccaagcctaacgacgtgtactccttcagcctggccagcagactgtacgccgaggaaagataccccatcctgcctgagtacctgcagtgcgtgaaagagctgtacagaggcggcctggaacctatcaacttccagacagccgccgaccaggccagagagctgatcaattcttgggtcgagagccagaccaacggcatcatcagaaacgtgctgcagcccagctccgtggattctcagacagccatggtgctggtcaacgccattgtgtttaaaggcctgtgggagaaaaccttcaaggacgaggacacccaggccatgcctttcagagtgacagagcaagagtccaagcctgtgcagatgatgtaccagatcggcctgtttagagtggcctccatggcctccgagaagatgaagatcctcgagctgcctttcgccagcggcaccatgtctatgctggtgctgctgcctgatgaggtgtccggactggaacagctcgagagcatcatcaacttcgagaagctgaccgagtggaccagcagcaacgtgatggaagaacggaagatcaaggtgtacctgcctcggatgaagatggaagagaagtacaacctgaccagcgtgctgatggctatgggcatcacagacgtgttctccagcagcgccaatctgagcggcatcagctctgccgagagcctgaagatttctcaggccgtgcatgctgcccacgccgagattaacgaagccggcagagaagttgtgggatctgccgaagcaggcgtggacgctgcttctgtgtctgaggaattccgggccgaccatccttttctgttctgcatcaagcacattgccaccaacgccgtgctgttctttggcagatgcgtgtccccttga

SEQ ID NO: 60 - DNA, 1503 bp, synthetic construct
  source 1..1503: mol_type = other DNA; note = VAMP3-OVA
atgagcacaggacctacagccgccacaggcagcaatagaaggctgcagcagacccagaaccaggtggacgaggtggtggacatcatgagagtgaacgtggacaaggtgctggaacgggaccagaagctgagcgagctggacgatagagccgatgctctgcaagctggcgcctctcagtttgagacatctgccgccaagctgaagcggaagtactggtggaagaactgcaagatgtgggccatcggcatcaccgtgctggtcatctttatcatcatcattatcgtgtgggtcgtgtcctctggcggcggaggatctggcggaggtggaagcggaggcggaggaagtggatctattggagccgccagcatggaattttgcttcgacgtgttcaaagaactgaaggtgcaccacgccaacgagaacatcttctactgccctatcgccatcatgagcgccctggctatggtgtatctgggcgccaaggacagcacccggacacagatcaacaaggtcgtcagattcgacaagctgcccggcttcggcgattctatcgaagcccagtgtggcaccagcgtgaacgtgcacagcagcctgagagacatcctgaatcagatcaccaagcctaacgacgtgtactccttcagcctggccagcagactgtacgccgaggaaagataccccatcctgcctgagtacctgcagtgcgtgaaagagctgtacagaggcggcctggaacctatcaacttccagacagccgccgaccaggccagagagctgatcaattcttgggtcgagagccagaccaacggcatcatcagaaacgtgctgcagcccagctccgtggattctcagacagccatggtgctggtcaacgccattgtgtttaaaggcctgtgggagaaaaccttcaaggacgaggacacccaggccatgcctttcagagtgacagagcaagagtccaagcctgtgcagatgatgtaccagatcggcctgtttagagtggcctccatggcctccgagaagatgaagatcctcgagctgcctttcgccagcggcaccatgtctatgctggtgctgctgcctgatgaggtgtccggactggaacagctcgagagcatcatcaacttcgagaagctgaccgagtggaccagcagcaacgtgatggaagaacggaagatcaaggtgtacctgcctcggatgaagatggaagagaagtacaacctgaccagcgtgctgatggctatgggcatcacagacgtgttctccagcagcgccaatctgagcggcatcagctctgccgagagcctgaagatttctcaggccgtgcatgctgcccacgccgagattaacgaagccggcagagaagttgtgggatctgccgaagcaggcgtggacgctgcttctgtgtctgaggaattccgggccgaccatccttttctgttctgcatcaagcacattgccaccaacgccgtgctgttctttggcagatgcgtgtccccttga

SEQ ID NO: 61 - DNA, 1626 bp, synthetic construct
  source 1..1626: mol_type = other DNA; note = VAMP4-OVA
atgcctccaaagttcaagcggcacctgaacgacgacgatgtgaccggctctgtgaagtccgagcggagaaacctgctggaagatgacagcgacgaggaagaggacttcttcctgcggggaccttctggccctagattcggccccagaaacgacaagatcaagcacgtgcagaaccaggtggacgaagtgatcgacgtgatgcaagagaacatcaccaaagtcatcgagcggggcgagagactggacgagctgcaggataagagcgagagcctgagcgataacgccaccgccttcagcaacagaagcaagcagctgcggagacagatgtggtggcggggctgcaagattaaggccatcatggctctggtggccgccatcctgctgctggtcatcatcatcctgatcgtgatgaagtaccggacaggcggcggaggatctggcggaggtggaagcggaggcggaggaagtggatctattggagccgccagcatggaattttgcttcgacgtgttcaaagaactgaaggtgcaccacgccaacgagaacatcttctactgccctatcgccatcatgagcgccctggctatggtgtatctgggcgccaaggacagcacccggacacagatcaacaaggtcgtcagattcgacaagctgcccggcttcggcgattctatcgaagcccagtgtggcaccagcgtgaacgtgcacagcagcctgagagacatcctgaatcagatcaccaagcctaacgacgtgtactccttcagcctggccagcagactgtacgccgaggaaagataccccatcctgcctgagtacctgcagtgcgtgaaagagctgtacagaggcggcctggaacctatcaacttccagacagccgccgaccaggccagagagctgatcaattcttgggtcgagagccagaccaacggcatcatcagaaacgtgctgcagcccagctccgtggattctcagacagccatggtgctggtcaacgccattgtgtttaaaggcctgtgggagaaaaccttcaaggacgaggacacccaggccatgcctttcagagtgacagagcaagagtccaagcctgtgcagatgatgtaccagatcggcctgtttagagtggcctccatggcctccgagaagatgaagatcctcgagctgcctttcgccagcggcaccatgtctatgctggtgctgctgcctgatgaggtgtccggactggaacagctcgagagcatcatcaacttcgagaagctgaccgagtggaccagcagcaacgtgatggaagaacggaagatcaaggtgtacctgcctcggatgaagatggaagagaagtacaacctgaccagcgtgctgatggctatgggcatcacagacgtgttctccagcagcgccaatctgagcggcatcagctctgccgagagcctgaagatttctcaggccgtgcatgctgcccacgccgagattaacgaagccggcagagaagttgtgggatctgccgaagcaggcgtggacgctgcttctgtgtctgaggaattccgggccgaccatccttttctgttctgcatcaagcacattgccaccaacgccgtgctgttctttggcagatgcgtgtccccttga

SEQ ID NO: 62 - DNA, 1503 bp, synthetic construct
  source 1..1503: mol_type = other DNA; note = VAMP8-OVA
atggaagaggctagtgaaggcggcggaaacgacagagtgcggaatctgcagtctgaggtggaaggcgtgaagaacatcatgacccagaacgtggaacggatcctggccagaggcgagaacctggaacacctgagaaacaagaccgaggacctggaagccaccagcgagcactttaagaccaccagccagaaggtggcccggaagttctggtggaagaatgtgaagatgatcgtgctgatctgcgtgatcgtgttcatcatcatcctgttcatcgtgctgttcgccaccggcgccttttctggcggcggaggatctggcggaggtggaagcggaggcggaggaagtggatctattggagccgccagcatggaattttgcttcgacgtgttcaaagaactgaaggtgcaccacgccaacgagaacatcttctactgccctatcgccatcatgagcgccctggctatggtgtatctgggcgccaaggacagcacccggacacagatcaacaaggtcgtcagattcgacaagctgcccggcttcggcgattctatcgaagcccagtgtggcaccagcgtgaacgtgcacagcagcctgagagacatcctgaatcagatcaccaagcctaacgacgtgtactccttcagcctggccagcagactgtacgccgaggaaagataccccatcctgcctgagtacctgcagtgcgtgaaagagctgtacagaggcggcctggaacctatcaacttccagacagccgccgaccaggccagagagctgatcaattcttgggtcgagagccagaccaacggcatcatcagaaacgtgctgcagcccagctccgtggattctcagacagccatggtgctggtcaacgccattgtgtttaaaggcctgtgggagaaaaccttcaaggacgaggacacccaggccatgcctttcagagtgacagagcaagagtccaagcctgtgcagatgatgtaccagatcggcctgtttagagtggcctccatggcctccgagaagatgaagatcctcgagctgcctttcgccagcggcaccatgtctatgctggtgctgctgcctgatgaggtgtccggactggaacagctcgagagcatcatcaacttcgagaagctgaccgagtggaccagcagcaacgtgatggaagaacggaagatcaaggtgtacctgcctcggatgaagatggaagagaagtacaacctgaccagcgtgctgatggctatgggcatcacagacgtgttctccagcagcgccaatctgagcggcatcagctctgccgagagcctgaagatttctcaggccgtgcatgctgcccacgccgagattaacgaagccggcagagaagttgtgggatctgccgaagcaggcgtggacgctgcttctgtgtctgaggaattccgggccgaccatccttttctgttctgcatcaagcacattgccaccaacgccgtgctgttctttggcagatgcgtgtccccttga

SEQ ID NO: 63 - DNA, 1899 bp, synthetic construct
  source 1..1899: mol_type = other DNA; note = VTI1B-OVA
atggctagctctgccgccagctctgagcacttcgagaagctgcacgagatcttcagaggcctgcacgaggacctgcagggcgttccagaaagactgctgggaacagccggcaccgaggaaaagaagaagctgatccgggacttcgacgagaagcagcaagaggccaatgagacactggccgagatggaagaggaactgagatacgcccctctgagcttcagaaaccccatgatgagcaagctgcggaactaccggaaggacctggccaagctgcatagagaagtgcggagcacccctctgacagctacacctggtggaagaggcgacatgaagtacggcatctacgccgtggaaaacgagcacatgaaccggctgcagagccagagagctatgctgctgcagggcaccgagagcctgaatagagccacacagagcatcgagcggagccacagaatcgccaccgagacagatcagatcggcagcgagatcatcgaggaactgggcgagcagagggaccagctggaaaggaccaagagcagactggtcaacaccagcgagaacctgagcaagagccggaagatcctgcggagcatgagcagaaaagtgaccaccaacaagctgctgctgagcatcatcatcctgctggaactggccatcctcggcggcctggtgtactacaagttcttcagaagccatggcggcggaggatctggcggaggtggaagcggaggcggaggaagtggatctattggagccgccagcatggaattttgcttcgacgtgttcaaagaactgaaggtgcaccacgccaacgagaacatcttctactgccctatcgccatcatgagcgccctggctatggtgtatctgggcgccaaggacagcacccggacacagatcaacaaggtcgtcagattcgacaagctgcccggcttcggcgattctatcgaagcccagtgtggcaccagcgtgaacgtgcacagcagcctgagagacatcctgaatcagatcaccaagcctaacgacgtgtactccttcagcctggccagcagactgtacgccgaggaaagataccccatcctgcctgagtacctgcagtgcgtgaaagagctgtacagaggcggcctggaacctatcaacttccagacagccgccgaccaggccagagagctgatcaattcttgggtcgagagccagaccaacggcatcatcagaaacgtgctgcagcccagctccgtggattctcagacagccatggtgctggtcaacgccattgtgtttaaaggcctgtgggagaaaaccttcaaggacgaggacacccaggccatgcctttcagagtgacagagcaagagtccaagcctgtgcagatgatgtaccagatcggcctgtttagagtggcctccatggcctccgagaagatgaagatcctcgagctgcctttcgccagcggcaccatgtctatgctggtgctgctgcctgatgaggtgtccggactggaacagctcgagagcatcatcaacttcgagaagctgaccgagtggaccagcagcaacgtgatggaagaacggaagatcaaggtgtacctgcctcggatgaagatggaagagaagtacaacctgaccagcgtgctgatggctatgggcatcacagacgtgttctccagcagcgccaatctgagcggcatcagctctgccgagagcctgaagatttctcaggccgtgcatgctgcccacgccgagattaacgaagccggcagagaagttgtgggatctgccgaagcaggcgtggacgctgcttctgtgtctgaggaattccgggccgaccatccttttctgttctgcatcaagcacattgccaccaacgccgtgctgttctttggcagatgcgtgtccccttga

SEQ ID NO: 64 - DNA, 1953 bp, synthetic construct
  source 1..1953: mol_type = other DNA; note = GOSR1-OVA
atggccgctggcacaagcagctactgggaagatctgcggaagcaggcccggcagctggaaaatgagctggacctgaagctggtgtccttcagcaagctgtgcaccagctacagccacagcagcaccagagatggcagacgggacagatacagcagcgacaccacacctctgctgaacggcagcagccaggaccggatgtttgagacaatggccatcgagatcgaacagctgctggccagactgaccggcgtgaacgataagatggccgagtacaccaactctgccggcgtgccaagtctgaacgccgctctgatgcacaccctgcagagacacagagacattctgcaggactacacccacgagttccacaagaccaaggccaacttcatggccattcgcgagcgcgagaatctgatgggctctgtgcggaaggacatcgagagctacaagagcggctctggcgtgaacaacagacggaccgagctgttcctgaaagagcacgaccacctgagaaacagcgaccggctgatcgaggaaaccatctctatcgccatggccaccaaagaaaacatgaccagccagcggggcatgctgaagtccatccacagcaagatgaacaccctggccaacagattccccgccgtgaacagcctgatccagcggatcaatctgagaaagcggcgggactctctgatcctcggcggagtgatcggcatctgtaccatcctgctgctgctctacgccttccatggcggcggaggatctggcggaggtggaagcggaggcggaggaagtggatctattggagccgccagcatggaattttgcttcgacgtgttcaaagaactgaaggtgcaccacgccaacgagaacatcttctactgccctatcgccatcatgagcgccctggctatggtgtatctgggcgccaaggacagcacccggacacagatcaacaaggtcgtcagattcgacaagctgcccggcttcggcgattctatcgaagcccagtgtggcaccagcgtgaacgtgcacagcagcctgagagacatcctgaatcagatcaccaagcctaacgacgtgtactccttcagcctggccagcagactgtacgccgaggaaagataccccatcctgcctgagtacctgcagtgcgtgaaagagctgtacagaggcggcctggaacctatcaacttccagacagccgccgaccaggccagagagctgatcaattcttgggtcgagagccagaccaacggcatcatcagaaacgtgctgcagcccagctccgtggattctcagacagccatggtgctggtcaacgccattgtgtttaaaggcctgtgggagaaaaccttcaaggacgaggacacccaggccatgcctttcagagtgacagagcaagagtccaagcctgtgcagatgatgtaccagatcggcctgtttagagtggcctccatggcctccgagaagatgaagatcctcgagctgcctttcgccagcggcaccatgtctatgctggtgctgctgcctgatgaggtgtccggactggaacagctcgagagcatcatcaacttcgagaagctgaccgagtggaccagcagcaacgtgatggaagaacggaagatcaaggtgtacctgcctcggatgaagatggaagagaagtacaacctgaccagcgtgctgatggctatgggcatcacagacgtgttctccagcagcgccaatctgagcggcatcagctctgccgagagcctgaagatttctcaggccgtgcatgctgcccacgccgagattaacgaagccggcagagaagttgtgggatctgccgaagcaggcgtggacgctgcttctgtgtctgaggaattccgggccgaccatccttttctgttctgcatcaagcacattgccaccaacgccgtgctgttctttggcagatgcgtgtccccttga

SEQ ID NO: 65 - DNA, 1557 bp, synthetic construct
  source 1..1557: mol_type = other DNA; note = BET1-OVA
atgcggagagccggacttggagaaggtgtccctcctggcaactacggcaattacggctacgccaacagcggctactctgcctgcgaggaagagaacgagagactgaccgagagcctgcggagcaaagtgaccgccatcaagagcctgagcatcgagatcggccacgaagtgaaaacccagaacaagctgctggccgagatggacagccagttcgacagcaccacaggctttctgggcaagaccatgggcaagctgaagatcctgagcagaggcagccagacaaagctgctgtgctacatgatgctgttcagcctgttcgtgttcttcatcatctactggatcatcaagctgagaggcggcggaggatctggcggaggtggaagcggaggcggaggaagtggatctattggagccgccagcatggaattttgcttcgacgtgttcaaagaactgaaggtgcaccacgccaacgagaacatcttctactgccctatcgccatcatgagcgccctggctatggtgtatctgggcgccaaggacagcacccggacacagatcaacaaggtcgtcagattcgacaagctgcccggcttcggcgattctatcgaagcccagtgtggcaccagcgtgaacgtgcacagcagcctgagagacatcctgaatcagatcaccaagcctaacgacgtgtactccttcagcctggccagcagactgtacgccgaggaaagataccccatcctgcctgagtacctgcagtgcgtgaaagagctgtacagaggcggcctggaacctatcaacttccagacagccgccgaccaggccagagagctgatcaattcttgggtcgagagccagaccaacggcatcatcagaaacgtgctgcagcccagctccgtggattctcagacagccatggtgctggtcaacgccattgtgtttaaaggcctgtgggagaaaaccttcaaggacgaggacacccaggccatgcctttcagagtgacagagcaagagtccaagcctgtgcagatgatgtaccagatcggcctgtttagagtggcctccatggcctccgagaagatgaagatcctcgagctgcctttcgccagcggcaccatgtctatgctggtgctgctgcctgatgaggtgtccggactggaacagctcgagagcatcatcaacttcgagaagctgaccgagtggaccagcagcaacgtgatggaagaacggaagatcaaggtgtacctgcctcggatgaagatggaagagaagtacaacctgaccagcgtgctgatggctatgggcatcacagacgtgttctccagcagcgccaatctgagcggcatcagctctgccgagagcctgaagatttctcaggccgtgcatgctgcccacgccgagattaacgaagccggcagagaagttgtgggatctgccgaagcaggcgtggacgctgcttctgtgtctgaggaattccgggccgaccatccttttctgttctgcatcaagcacattgccaccaacgccgtgctgttctttggcagatgcgtgtccccttga

SEQ ID NO: 66 - DNA, 2073 bp, synthetic construct
  source 1..2073: mol_type = other DNA; note = BET1L-OVA
atggccttttgcgccatcctgctggtgcctagcctgtgcagaatgcccagcctgcctacaagcccttgggcctttcctgtgcattgggccggcttcatgttcaagcccctggactggcagggcaacgacttcttcccacctcaagacgaagtgctggccccttgcctgggcatcaagacacctctgaagcacgagccctgtgctagcctgcctttcagcgtgctgtttcagagcagcgccagccagtctctgctgggcacaatgggatctctgagccctcacctgtgcggccacacaatgtgccctgtgaatcctgagctgccactgagcttccaggccgaccatagatctgcccagccagatgcctgcagtcccctgtgtcatccatctagcctgctgcctagcttccacaccgcttctctgcccttcagcattcacgcccaccactctccactgccttgcgaccttgatcctcctctgtacctggccgagacagtgtccctgctggaagaatggggacctcctagcagctgccccatgcagtgcaagctgacatctcaccctgccagactgacccatctgcctccatgtctgtggggctttgccgtggctctgaagccttcttgggctggccttgctccttctctgctgcctccacctagaatgagcctgtgtagacccctgtccttcctgcggcatcagtgtccttggctgccttggcaggctcaccaaggacttgttccttggagcccctctatggtggccgctgcctgtatcgtgtctcctagcggacactgtagatgccagcctttcatccctcacgtgttcctcggacacggcggcctgacatctgtgtctggcgaatgcggaggcggcggaggatctggcggaggtggaagcggaggcggaggaagtggatctattggagccgccagcatggaattttgcttcgacgtgttcaaagaactgaaggtgcaccacgccaacgagaacatcttctactgccctatcgccatcatgagcgccctggctatggtgtatctgggcgccaaggacagcacccggacacagatcaacaaggtcgtcagattcgacaagctgcccggcttcggcgattctatcgaagcccagtgtggcaccagcgtgaacgtgcacagcagcctgagagacatcctgaatcagatcaccaagcctaacgacgtgtactccttcagcctggccagcagactgtacgccgaggaaagataccccatcctgcctgagtacctgcagtgcgtgaaagagctgtacagaggcggcctggaacctatcaacttccagacagccgccgaccaggccagagagctgatcaattcttgggtcgagagccagaccaacggcatcatcagaaacgtgctgcagcccagctccgtggattctcagacagccatggtgctggtcaacgccattgtgtttaaaggcctgtgggagaaaaccttcaaggacgaggacacccaggccatgcctttcagagtgacagagcaagagtccaagcctgtgcagatgatgtaccagatcggcctgtttagagtggcctccatggcctccgagaagatgaagatcctcgagctgcctttcgccagcggcaccatgtctatgctggtgctgctgcctgatgaggtgtccggactggaacagctcgagagcatcatcaacttcgagaagctgaccgagtggaccagcagcaacgtgatggaagaacggaagatcaaggtgtacctgcctcggatgaagatggaagagaagtacaacctgaccagcgtgctgatggctatgggcatcacagacgtgttctccagcagcgccaatctgagcggcatcagctctgccgagagcctgaagatttctcaggccgtgcatgctgcccacgccgagattaacgaagccggcagagaagttgtgggatctgccgaagcaggcgtggacgctgcttctgtgtctgaggaattccgggccgaccatccttttctgttctgcatcaagcacattgccaccaacgccgtgctgttctttggcagatgcgtgtccccttga

SEQ ID NO: 67 - DNA, 1848 bp, synthetic construct
  source 1..1848: mol_type = other DNA; note = SEC22B-OVA
atggtcctgctgaccatgattgccagagtggccgatggactgcctctggccgctagcatgcaagaggatgagcagagcggcagagatctgcagcagtaccagtctcaggccaagcagctgttccggaagctgaacgagcagagccctaccagatgcacccttgaagccggcgctatgaccttccactacatcatcgagcagggcgtgtgctacctggtgctgtgcgaagccgcctttcctaagaagctggccttcgcctacctggaagatctgcacagcgagttcgatgagcagcacggcaagaaggtgcccaccgtcagcagaccctacagcttcatcgagttcgacaccttcatccaaaagaccaagaagctgtacatcgacagccgggccagaagaaacctgggcagcatcaataccgagctgcaggacgtgcagagaatcatggtggccaacatcgaggaagtgctgcagagaggcgaagccctgtctgccctggatagcaaggccaacaatctgagcagcctgagcaagaagtaccggcaggacgccaagtacctgaacatgagaagcacctacgccaagctggccgccgtggccgtgttcttcatcatgctgatcgtgtacgtgcggttctggtggcttggcggcggaggatctggcggaggtggaagcggaggcggaggaagtggatctattggagccgccagcatggaattttgcttcgacgtgttcaaagaactgaaggtgcaccacgccaacgagaacatcttctactgccctatcgccatcatgagcgccctggctatggtgtatctgggcgccaaggacagcacccggacacagatcaacaaggtcgtcagattcgacaagctgcccggcttcggcgattctatcgaagcccagtgtggcaccagcgtgaacgtgcacagcagcctgagagacatcctgaatcagatcaccaagcctaacgacgtgtactccttcagcctggccagcagactgtacgccgaggaaagataccccatcctgcctgagtacctgcagtgcgtgaaagagctgtacagaggcggcctggaacctatcaacttccagacagccgccgaccaggccagagagctgatcaattcttgggtcgagagccagaccaacggcatcatcagaaacgtgctgcagcccagctccgtggattctcagacagccatggtgctggtcaacgccattgtgtttaaaggcctgtgggagaaaaccttcaaggacgaggacacccaggccatgcctttcagagtgacagagcaagagtccaagcctgtgcagatgatgtaccagatcggcctgtttagagtggcctccatggcctccgagaagatgaagatcctcgagctgcctttcgccagcggcaccatgtctatgctggtgctgctgcctgatgaggtgtccggactggaacagctcgagagcatcatcaacttcgagaagctgaccgagtggaccagcagcaacgtgatggaagaacggaagatcaaggtgtacctgcctcggatgaagatggaagagaagtacaacctgaccagcgtgctgatggctatgggcatcacagacgtgttctccagcagcgccaatctgagcggcatcagctctgccgagagcctgaagatttctcaggccgtgcatgctgcccacgccgagattaacgaagccggcagagaagttgtgggatctgccgaagcaggcgtggacgctgcttctgtgtctgaggaattccgggccgaccatccttttctgttctgcatcaagcacattgccaccaacgccgtgctgttctttggcagatgcgtgtccccttga

SEQ ID NO: 68 - DNA, 1980 bp, synthetic construct
  source 1..1980: mol_type = other DNA; note = USE1-OVA
atggccgcctctagactggaactgaatctcgtgcggctgctgagcagatgcgaagctatggccgccgagaagagggaccctgatgaatggcggctcgagaaatatgtgggcgccctggaagatatgctgcaggccctgaaagtgcacgccagcaagcctgccagcgaagtgatcaacgagtacagctggaaggtggacttcctgaagggcatgctccaggccgagaagctgacaagcagctctgaaaaggccctggccaaccagtttctggcccctggtagagtgcctaccaccgccagagaaagagtgccagccaccaagacagtgcacctccagagcagagccagatacaccagcgagatgagaagcgagctgctgggcacagattctgccgagcctgaaatggacgtgcggaagagaacaggcgtggcaggctctcagcctgtgtccgaaaaacagctggccgctgagctggatctggtgctgcagagacaccagaacctgcaagagaagctggccgaggaaatgctgggcctcgccagatctctgaaaacaaacaccctggccgctcagagcgtgatcaagaaggacaatcagaccctgagccacagcctgaagatggccgaccagaatctggaaaagctgaaaaccgagagcgagcggctggaacagcacacccagaaaagcgtgaactggctgctgtgggccatgctgatcatcgtgtgcttcatcttcatcagcatgatcctgttcatccggatcatgcccaagctgaaaggcggcggaggatctggcggaggtggaagcggaggcggaggaagtggatctattggagccgccagcatggaattttgcttcgacgtgttcaaagaactgaaggtgcaccacgccaacgagaacatcttctactgccctatcgccatcatgagcgccctggctatggtgtatctgggcgccaaggacagcacccggacacagatcaacaaggtcgtcagattcgacaagctgcccggcttcggcgattctatcgaagcccagtgtggcaccagcgtgaacgtgcacagcagcctgagagacatcctgaatcagatcaccaagcctaacgacgtgtactccttcagcctggccagcagactgtacgccgaggaaagataccccatcctgcctgagtacctgcagtgcgtgaaagagctgtacagaggcggcctggaacctatcaacttccagacagccgccgaccaggccagagagctgatcaattcttgggtcgagagccagaccaacggcatcatcagaaacgtgctgcagcccagctccgtggattctcagacagccatggtgctggtcaacgccattgtgtttaaaggcctgtgggagaaaaccttcaaggacgaggacacccaggccatgcctttcagagtgacagagcaagagtccaagcctgtgcagatgatgtaccagatcggcctgtttagagtggcctccatggcctccgagaagatgaagatcctcgagctgcctttcgccagcggcaccatgtctatgctggtgctgctgcctgatgaggtgtccggactggaacagctcgagagcatcatcaacttcgagaagctgaccgagtggaccagcagcaacgtgatggaagaacggaagatcaaggtgtacctgcctcggatgaagatggaagagaagtacaacctgaccagcgtgctgatggctatgggcatcacagacgtgttctccagcagcgccaatctgagcggcatcagctctgccgagagcctgaagatttctcaggccgtgcatgctgcccacgccgagattaacgaagccggcagagaagttgtgggatctgccgaagcaggcgtggacgctgcttctgtgtctgaggaattccgggccgaccatccttttctgttctgcatcaagcacattgccaccaacgccgtgctgttctttggcagatgcgtgtccccttga

SEQ ID NO: 69 - DNA, 1881 bp, synthetic construct
  source 1..1881: mol_type = other DNA; note = VAMP7-pc-OVA
atggccatcctgttcgccgtggtggctagaggcacaaccattctggccaagcacgcttggtgcggcggcaactttctggaagtgaccgagcagatcctggccaagattcccagcgagaacaacaagctgacctacagccacggcaactacctgttccactacatctgccaggaccggatcgtgtacctgtgcatcaccgacgacgacttcgagcggagcagagccttcaacttcctgaacgagatcaagaagcggttccagaccacctacggcagcagagcacaaacagccctgccttacgccatgaacagcgagttcagctctgtgctggccgctcagctgaagcaccactccgagaacaaaggcctggacaaagtgatggaaacacaggcccaggtggacgagctgaagggcatcatggtccgaaacatcgacctggtggcccagagaggcgagagactggaactgctgatcgacaagaccgagaacctggtggacagcagcgtgaccttcaagaccaccagcagaaacctggccagagccatgtgcatgaagaacctgaagctgacgatcatcatcattatcgtgtccatcgtgttcatctacatcatcgtgtccccactgtgtggcggcttcacctggcctagctgtgtgaagaaatctggcggcggaggatctggcggaggtggaagcggaggcggtggatctagaagggccagaagaggatctatcggagccgccagcatggaattttgcttcgacgtgttcaaagaactgaaggtgcaccacgccaacgagaacatcttctactgccctatcgccatcatgagcgccctggctatggtgtatctgggcgccaaggacagcacccggacacagatcaacaaggtcgtcagattcgacaagctgcccggcttcggcgattctatcgaagcccagtgtggcaccagcgtgaacgtgcacagcagcctgagagacatcctgaatcagatcaccaagcctaacgacgtgtactccttcagcctggccagcagactgtacgccgaggaaagataccccatcctgcctgagtacctgcagtgcgtgaaagagctgtacagaggcggcctggaacctatcaacttccagacagccgccgaccaggccagagagctgatcaattcttgggtcgagagccagaccaacggcatcatcagaaacgtgctgcagcccagctccgtggattctcagacagccatggtgctggtcaacgccattgtgtttaaaggcctgtgggagaaaaccttcaaggacgaggacacccaggccatgcctttcagagtgacagagcaagagtccaagcctgtgcagatgatgtaccagatcggcctgtttagagtggcctccatggcctccgagaagatgaagatcctcgagctgcctttcgccagcggcaccatgtctatgctggtgctgctgcctgatgaggtgtccggactggaacagctcgagagcatcatcaacttcgagaagctgaccgagtggaccagcagcaacgtgatggaagaacggaagatcaaggtgtacctgcctcggatgaagatggaagagaagtacaacctgaccagcgtgctgatggctatgggcatcacagacgtgttctccagcagcgccaatctgagcggcatcagctctgccgagagcctgaagatttctcaggccgtgcatgctgcccacgccgagattaacgaagccggcagagaagttgtgggatctgccgaagcaggcgtggacgctgcttctgtgtctgaggaattccgggccgaccatccttttctgttctgcatcaagcacattgccaccaacgccgtgctgttctttggcagatgcgtgtccccttga

SEQ ID NO: 70 - DNA, 2409 bp, synthetic construct
  source 1..2409: mol_type = other DNA; note = LAMP[OVA]
atggctgcccctggctctgctagaaggcctctgctgttgctgcttctgctgctgctcctgggcctgatgcattgtgcctctgccgccatgttcatggtcaagaacggcaatggcaccgcctgcatcatggccaatttcagcgccgccttcagcgtgaactacgacaccaagagcggccccaagaacatgaccttcgacctgccttctgacgccaccgtggtgctgaatagaagcagctgcggcaaagagaacaccagcgatcccagcctcgtgatcgcctttggcagaggccatacactgaccctgaacttcacccggaacgccaccagatacagcgtgcagctgatgagcttcgtgtacaacctgagcgacacccatctgttccccaacgccagcagcaaagagatcaagaccgtcgagagcatcaccgacatccgggccgacatcgacaaaaagtacagatgcgtgtccggcacacaggtgcacatgaacaacgtgaccgtgacactgcacgacgccaccatccaggcctacctgagcaacagctctttcagcaggggcgagacaagatgcgagcaggacagaccctctcctaccactgctcctccagctccaccttctccaagtccatctcctgtgcctaagagccccagcgtggacaagtacaatgtgtctggcaccaacggcacctgtctgctggcttctatgggcctgcagctgaacctgacctacgagcggaaggacaacaccaccgtgaccagactgctgaacatcaaccccaacaagaccagcgccagcggatcttgtggcgcccatctggttacactggaactgcacagcgagggcaccacagtgctgctgttccagttcggcatgaacgccagctccagccggttcttcctgcaaggcatccagctgaacaccatcctgcctgacgccagagatcctgccttcaaggccgccaatggaagcctgagagcactgcaggccacagtgggcaacagctacaagtgcaacgccgaggaacacgtgcgcgtgaccaaggccttctccgtgaacatcttcaaagtgtgggtgcaagcctttaaggtggaaggcggccagtttggcagcgtggaagaatgcctgctggacgagaatagcatgggctctatcggagccgccagcatggaattttgcttcgacgtgttcaaagagctgaaggtccaccacgccaacgagaatatcttctactgccctatcgccatcatgagcgccctggccatggtgtatctgggcgccaaggatagcacccggacacagatcaacaaggtcgtcagattcgacaagctgcccggcttcggcgattctatcgaagcccagtgtggcacctccgtgaatgtgcacagcagcctgagggacatcctgaaccagatcaccaagcctaacgacgtgtacagcttcagcctggcctccagactgtacgccgaagagagataccccattctgcccgagtacctgcagtgtgtgaaagaactgtacagaggcggcctggaacctatcaacttccagacagccgccgaccaggccagagagctgatcaattcttgggtcgagagccagaccaatggcatcatccggaacgtgctgcagcccagctctgtggattctcagactgccatggtgctggtcaacgccatcgtgtttaaaggcctgtgggagaaaaccttcaaggacgaggacacccaggccatgcctttcagagtgaccgagcaagagtccaagcctgtgcagatgatgtaccagatcggcctgtttagagtggcctccatggcctccgagaagatgaagatcctcgagctgcctttcgccagcggcaccatgtctatgttggtgctgctgcccgatgaggtgtccggactggaacaactggaatccatcatcaacttcgagaagctgaccgagtggaccagctccaacgtgatggaagaacggaagatcaaggtgtacctgcctcggatgaagatggaagagaagtacaatctgaccagcgtgctgatggccatgggaatcaccgatgtgttctccagcagcgccaacctgtctggcatcagctctgccgagagcctgaagatttctcaggccgtgcatgccgctcacgccgagatcaatgaagccggcagagaagttgtgggatctgccgaagcaggcgtggacgctgcatctgtgtctgaggaattcagagccgaccatccttttctgttctgcatcaagcacattgccaccaacgccgtgctgttcttcggaagatgtgtgtcccctctgatcccaatcgccgttggaggtgctctggctggactggtgctgatcgtgctgattgcctacctcgtgggcagaaagagaagccacgccggctaccagaccatctga

SEQ ID NO: 71 - DNA, 753 bp, Homo sapiens
  source 1..753: mol_type = genomic DNA
atggcggcagggaccagcagttactgggaagatctcaggaaacaggctcgacagctggaaaatgaacttgacctgaaactagtttccttcagcaaactatgtacaagttacagtcatagcagtacccgagatggaagacgcgacaggtatagttctgatacaacaccccttttaaatggatcaagccaagacagaatgtttgagacaatggcgattgagattgaacaacttttggcaaggcttacaggggtaaatgataaaatggcagaatataccaacagtgcaggtgtcccctccttgaatgcagccctgatgcatacattacagcggcatagagacatattgcaggattatacacatgaattccataaaaccaaagcaaactttatggcaatacgggaaagggagaatcttatgggatcagtacgaaaagatattgagtcatataaaagtgggtctggagtaaacaacagaagaactgagctatttttgaaagaacatgaccaccttcgaaactcagatcgtctgatagaagagacaataagcattgctatggcaacaaaagaaaatatgacttcacagagaggaatgttgaagtcaattcacagcaaaatgaacactttggccaatcgttttcctgctgtaaacagcctgatccagaggatcaacctgaggaagcggcgggactcgctcatcctagggggtgttattgggatctgtaccatcctgttgctgctgtatgcgttccattga

SEQ ID NO: 72 - DNA, 711 bp, Homo sapiens
  source 1..711: mol_type = genomic DNA
atggcaccggacccctggttctccacatacgattctacttgtcaaattgcccaagaaattgctgagaaaattcaacaacgaaatcaatatgaaagaaaaggtgaaaaggcaccaaagcttaccgtgacaatcagagctttgttgcagaacctgaaggaaaagatcgcccttttgaaggacttattgctaagagctgtgtcaacacatcagataacacagcttgaaggggaccgaagacagaacctcttggatgatcttgtaactcgagagagactacttctggcatcctttaagaatgagggtgccgaaccagatctaatcaggtccagcctgatgagtgaagaggctaagcgaggagcacccaacccttggctctttgaggagccagaggagaccagaggcttgggttttgatgaaatccggcaacagcagcagaaaattatccaagaacaggacgcaggccttgatgccctttcctctatcataagtcgccaaaaacaaatggggcaggaaattgggaatgaattggatgaacaaaatgagataattgacgaccttgccaacctagtggagaacacagatgaaaaacttcgcaatgaaaccaggcgggtaaacatggtggacagaaagtcagcctcttgtgggatgatcatggtgattttactgctgcttgtggctatcgtggttgttgcagtctggccgaccaactga

SEQ ID NO: 73 - DNA, 831 bp, Homo sapiens
  source 1..831: mol_type = genomic DNA
atgtcatacggtcccttagacatgtaccggaacccggggccctcggggccccagctccgggacttcagcagcatcatccagacgtgcagcggcaacatccagcggatcagccaagccactgctcagataaagaatttgatgagccagctaggaactaagcaggactcaagcaagctacaggaaaatctgcaacagttacaacactccacaaatcagctcgccaaggaaacaaatgaattgctgaaagaattagggtccttgccccttcccttatctacttcagaacagcgccagcagagacttcagaaggaacgcctcatgaatgacttctctgcagccttaaacaatttccaggctgtgcagagaagggtatctgaaaaggaaaaggagagtattgccagagcaagagctggatctcgtctttctgcagaagagaggcaaagagaggagcagctggtctcatttgacagccatgaggagtggaaccagatgcagagccaggaggatgaggtggccatcactgagcaggatttggaacttattaaagaaagagaaacggcaattcggcagctggaggctgacattttggatgtcaatcagatatttaaagatttggccatgatgatccatgaccagggtgatctgattgatagcatagaagccaatgtggaaagctcagaggtgcacgtcgaaagagccactgaacagttacagcgagctgcttactatcagaaaaaatctcgcaagaagatgtgtatcctggtgcttgtcctgtcagtgattattctaatcttgggacttattatctggctagtttataaaacgaagtga

SEQ ID NO: 74 - DNA, 303 bp, Homo sapiens
  source 1..303: mol_type = genomic DNA
atggaggaagccagtgaaggtggaggaaatgatcgtgtgcggaacctgcaaagtgaggtggagggagttaagaatattatgacccagaatgtggagcggatcctggcccggggggaaaacttggaacatctccgcaacaagacagaggatctggaagccacatctgagcacttcaagacgacatcgcagaaggtggctcgaaaattctggtggaagaacgtgaagatgattgtccttatctgcgtgattgtttttatcatcatcctcttcattgtgctctttgccactggtgccttctcttaa

SEQ ID NO: 75 - DNA, 648 bp, Homo sapiens
  source 1..648: mol_type = genomic DNA
atggtgttgctaacaatgatcgcccgagtggcggacgggctcccgctggccgcctcgatgcaggaggacgaacagtctggccgggaccttcaacaatatcagagtcaggctaagcaactctttcgaaagttgaatgaacagtcccctaccagatgtaccttggaagcaggagccatgacttttcactacattattgagcagggggtgtgttatttggttttatgtgaagctgccttccctaagaagttggcttttgcctacctagaagatttgcactcagaatttgatgaacagcatggaaagaaggtgcccactgtgtcccgaccctattcctttattgaatttgatactttcattcagaaaaccaagaagctctacattgacagtcgtgctcgaagaaatctaggctccatcaacactgaattgcaagatgtgcagaggatcatggtggccaatattgaagaagtgttacaacgaggagaagcactctcagcattggattcaaaggctaacaatttgtccagtctgtccaagaaataccgccaggatgcgaagtacttgaacatgcgttccacttatgccaaacttgcagcagtagctgtatttttcatcatgttaatagtgtatgtccgattctggtggctgtga

SEQ ID NO: 76 - DNA, 768 bp, Homo sapiens
  source 1..768: mol_type = genomic DNA
atgtccatggaggaccccttctttgtggtgaaaggagaggtacagaaagcagtcaacactgcccagggattgtttcagagatggacagagctcctccaggacccctccacagcaacaagggaagaaatcgactggaccaccaacgagctgagaaataacctccggagcatagagtgggatctagaggaccttgatgaaaccatcagcatagttgaagcaaatcctagaaaatttaaccttgatgcaactgaattgagtataagaaaagccttcattacaagtactcggcaagttgtcagggacatgaaagatcagatgtcaacttcatctgtgcaggcattagctgaaagaaaaaatagacaggcactgctgggagacagtggcagccagaactggagcactggaacaacagataaatatgggcgtctggaccgagagctccagagagccaattctcatttcattgaggagcagcaggcacagcagcagttgatcgtggaacagcaggatgagcagttggagctggtctctggcagcatcggggtgctgaagaacatgtcccagcgcatcggaggggagctggaggaacaggcagttatgttggaagatttctctcacgaattggagagcactcagtcccggctggacaatgtgatgaagaaacttgcaaaagtatctcatatgaccagtgatcggcgccaatggtgtgccatagccatcctctttgcagtcctgttggttgtgctcatcctcttcttagtgctgtga

SEQ ID NO: 77 - DNA, 303 bp, Homo sapiens
  source 1..303: mol_type = genomic DNA
atgtctacaggtccaactgctgccactggcagtaatcgaagacttcagcagacacaaaatcaagtagatgaggtggtggacataatgcgagttaacgtggacaaggttctggaaagagaccagaagctctctgagttagacgaccgtgcagacgcactgcaggcaggcgcttctcaatttgaaacgagcgcagccaagttgaagaggaaatattggtggaagaattgcaagatgtgggcaatcgggattactgttctggttatcttcatcatcatcatcatcgtgtgggttgtctcttcatga

SEQ ID NO: 78 - DNA, 426 bp, Homo sapiens
  source 1..426: mol_type = genomic DNA
atgcctcccaagtttaagcgccacctcaatgatgatgatgtcacaggttctgtgaaaagtgaaaggagaaatcttttggaagatgattcagatgaagaagaggacttttttctaaggggaccatctggaccaagatttggacctagaaatgataaaattaagcatgttcagaatcaagtggatgaagttattgatgtcatgcaagaaaatattacaaaggtaattgagagaggggagagactagatgaactacaggacaaatcagaaagcttatcggataatgcaacagcttttagcaacagatccaaacaacttcgaaggcaaatgtggtggcgtggatgcaaaataaaagccatcatggctttggttgctgctatccttttgctagtgattatcattcttatagtcatgaaataccgtacttga

SEQ ID NO: 79 - DNA, 699 bp, Homo sapiens
  source 1..699: mol_type = genomic DNA
atggcctcctccgccgcctcctcggagcatttcgagaagctgcacgagatcttccgcggcctccatgaagacctacaaggggtgcccgagcggctgctggggacggcggggaccgaagaaaagaagaaattgatcagggattttgatgaaaagcaacaggaagcaaatgaaacgctggcagagatggaggaggagctacgttatgcacccctgtctttccgaaaccccatgatgtctaagcttcgaaactaccggaaggaccttgctaaactccatcgggaggtgagaagcacacctttgacagccacacctggaggccgaggagacatgaaatatggcatatatgctgtagagaatgagcatatgaatcggctacagtctcaaagggcaatgcttctgcagggcactgaaagcctgaaccgggccacccaaagtattgaacgttctcatcggattgccacagagactgaccagattggctcagaaatcatagaagagctgggggaacaacgagaccagttagaacgtaccaagagtagactggtaaacacaagtgaaaacttgagcaaaagtcggaagattctccgttcaatgtccagaaaagtgacaaccaacaagctgctgctttccattatcatcttactggagctcgccatcctgggaggcctggtttactacaaattctttcgcagccattga

SEQ ID NO: 80 - DNA, 357 bp, Homo sapiens
  source 1..357: mol_type = genomic DNA
atgaggcgtgcaggcctgggtgaaggagtacctcctggcaactatgggaactatggctatgctaatagtgggtatagtgcctgtgaagaagaaaatgagaggctcactgaaagtctgagaagcaaagtaactgctataaaatctctttccattgaaataggccatgaagttaaaacccagaataaattattagctgaaatggattcacaatttgattccacaactggatttctaggtaaaactatgggcaaactgaagattttatccagagggagccaaacaaagctgctgtgctatatgatgctgttttctttatttgtcttttttatcatttattggattattaaactgaggtga

SEQ ID NO: 81 - DNA, 873 bp, Homo sapiens
  source 1..873: mol_type = genomic DNA
atggcattctgtgccatcctccttgtccccagcctctgcaggatgccctccttacccacctctccctgggccttccctgtccactgggctggattcatgttcaaaccactggactggcagggcaacgacttcttcccacctcaagatgaggtcctcgccccttgtcttggcataaaaacacctttaaagcatgagccatgtgcttctttgcccttttctgtcctgttccaatcttctgcctcccagtcactcctggggactatgggatcactgtccccccacctgtgtggccacaccatgtgtcctgtcaatccagaactgcctctgagcttccaggctgaccacagatcagcacagcctgatgcctgcagcccactttgtcacccttcctcccttcttccttccttccacacagcaagcctacctttctccatccatgctcaccatagcccccttccttgtgacctggaccctccattgtacctggctgagactgtcagcctcctggaggagtggggtccaccttcttcttgccctatgcagtgcaagctcacttctcacccagcaaggttgactcatctgcctccatgtctctggggctttgctgttgccctgaaacctagctgggctggtcttgctcccagcttgcttccccctcctcggatgtccctttgcaggcccctgtcgttcctccggcaccagtgtccttggctgccatggcaagctcatcaggggcttgtaccctggtcaccaagcatggtagcagctgcctgcattgtatctccatctggtcactgcaggtgccaacccttcatcccccatgttttcctgggccatggagggctgacctccgtttctggggaatgtggctga

SEQ ID NO: 82 - DNA, 780 bp, Homo sapiens
  source 1..780: mol_type = genomic DNA
atggcggcgtcgaggctggagctaaacctggtgcggctgctatcccgctgcgaggcgatggcagcggagaaacgggacccggacgagtggcgcctggagaagtacgtgggagccctagaggacatgttgcaggccctgaaggtccacgcgagcaaaccggcctctgaggtgatcaatgaatattcctggaaggtggattttctgaaggggatgctgcaagccgagaagctgacctcctcctcagagaaagcactggccaaccagttcctggcccctggccgtgtgccaaccacagccagagagcgagtgcccgccacaaagacggtgcatctgcagtcacgggcgcggtacaccagcgagatgcggagtgagctactaggcacggactctgcagagcctgagatggacgtaaggaagagaactggagtggcagggtcccagccagtgagtgagaagcagttggcagctgagctagacctcgtcctgcagcgacatcagaacctccaggaaaagctggcggaagagatgctaggactggcccggagcctcaagaccaataccctggccgcccagagtgtcatcaagaaggacaaccagaccctgtcacactcactgaaaatggcggaccagaacctggagaaactgaagacggagtcagagcgtctggagcagcacacgcagaagtcagtcaactggctgctctgggccatgctcattatcgtctgcttcatcttcattagcatgatcctcttcattcgaatcatgcctaaactcaaataa

SEQ ID NO: 83 - protein, 250 aa, Homo sapiens
MAAGTSSYWEDLRKQARQLENELDLKLVSFSKLCTSYSHSSTRDGRRDRYSSDTTPLLNGSSQDRMFETMAIEIEQLLARLTGVNDKMAEYTNSAGVPSLNAALMHTLQRHRDILQDYTHEFHKTKANFMAIRERENLMGSVRKDIESYKSGSGVNNRRTELFLKEHDHLRNSDRLIEETISIAMATKENMTSQRGMLKSIHSKMNTLANRFPAVNSLIQRINLRKRRDSLILGGVIGICTILLLLYAFH

SEQ ID NO: 84 - protein, 236 aa, Homo sapiens
MAPDPWFSTYDSTCQIAQEIAEKIQQRNQYERKGEKAPKLTVTIRALLQNLKEKIALLKDLLLRAVSTHQITQLEGDRRQNLLDDLVTRERLLLASFKNEGAEPDLIRSSLMSEEAKRGAPNPWLFEEPEETRGLGFDEIRQQQQKIIQEQDAGLDALSSIISRQKQMGQEIGNELDEQNEIIDDLANLVENTDEKLRNETRRVNMVDRKSASCGMIMVILLLLVAIVVVAVWPTN

SEQ ID NO: 85 - protein, 276 aa, Homo sapiens
MSYGPLDMYRNPGPSGPQLRDFSSIIQTCSGNIQRISQATAQIKNLMSQLGTKQDSSKLQENLQQLQHSTNQLAKETNELLKELGSLPLPLSTSEQRQQRLQKERLMNDFSAALNNFQAVQRRVSEKEKESIARARAGSRLSAEERQREEQLVSFDSHEEWNQMQSQEDEVAITEQDLELIKERETAIRQLEADILDVNQIFKDLAMMIHDQGDLIDSIEANVESSEVHVERATEQLQRAAYYQKKSRKKMCILVLVLSVIILILGLIIWLVYKTK

SEQ ID NO: 86 - protein, 100 aa, Homo sapiens
MEEASEGGGNDRVRNLQSEVEGVKNIMTQNVERILARGENLEHLRNKTEDLEATSEHFKTTSQKVARKFWWKNVKMIVLICVIVFIIILFIVLFATGAFS

SEQ ID NO: 87 - protein, 215 aa, Homo sapiens
MVLLTMIARVADGLPLAASMQEDEQSGRDLQQYQSQAKQLFRKLNEQSPTRCTLEAGAMTFHYIIEQGVCYLVLCEAAFPKKLAFAYLEDLHSEFDEQHGKKVPTVSRPYSFIEFDTFIQKTKKLYIDSRARRNLGSINTELQDVQRIMVANIEEVLQRGEALSALDSKANNLSSLSKKYRQDAKYLNMRSTYAKLAAVAVFFIMLIVYVRFWWL

SEQ ID NO: 88 - protein, 255 aa, Homo sapiens
MSMEDPFFVVKGEVQKAVNTAQGLFQRWTELLQDPSTATREEIDWTTNELRNNLRSIEWDLEDLDETISIVEANPRKFNLDATELSIRKAFITSTRQVVRDMKDQMSTSSVQALAERKNRQALLGDSGSQNWSTGTTDKYGRLDRELQRANSHFIEEQQAQQQLIVEQQDEQLELVSGSIGVLKNMSQRIGGELEEQAVMLEDFSHELESTQSRLDNVMKKLAKVSHMTSDRRQWCAIAILFAVLLVVLILFLVL

SEQ ID NO: 89 - protein, 100 aa, Homo sapiens
MSTGPTAATGSNRRLQQTQNQVDEVVDIMRVNVDKVLERDQKLSELDDRADALQAGASQFETSAAKLKRKYWWKNCKMWAIGITVLVIFIIIIIVWVVSS

SEQ ID NO: 90 - protein, 141 aa, Homo sapiens
MPPKFKRHLNDDDVTGSVKSERRNLLEDDSDEEEDFFLRGPSGPRFGPRNDKIKHVQNQVDEVIDVMQENITKVIERGERLDELQDKSESLSDNATAFSNRSKQLRRQMWWRGCKIKAIMALVAAILLLVIIILIVMKYRT

SEQ ID NO: 91 - protein, 232 aa, Homo sapiens
MASSAASSEHFEKLHEIFRGLHEDLQGVPERLLGTAGTEEKKKLIRDFDEKQQEANETLAEMEEELRYAPLSFRNPMMSKLRNYRKDLAKLHREVRSTPLTATPGGRGDMKYGIYAVENEHMNRLQSQRAMLLQGTESLNRATQSIERSHRIATETDQIGSEIIEELGEQRDQLERTKSRLVNTSENLSKSRKILRSMSRKVTTNKLLLSIIILLELAILGGLVYYKFFRSH

SEQ ID NO: 92 - protein, 118 aa, Homo sapiens
MRRAGLGEGVPPGNYGNYGYANSGYSACEEENERLTESLRSKVTAIKSLSIEIGHEVKTQNKLLAEMDSQFDSTTGFLGKTMGKLKILSRGSQTKLLCYMMLFSLFVFFIIYWIIKLR

SEQ ID NO: 93 - protein, 290 aa, Homo sapiens
MAFCAILLVPSLCRMPSLPTSPWAFPVHWAGFMFKPLDWQGNDFFPPQDEVLAPCLGIKTPLKHEPCASLPFSVLFQSSASQSLLGTMGSLSPHLCGHTMCPVNPELPLSFQADHRSAQPDACSPLCHPSSLLPSFHTASLPFSIHAHHSPLPCDLDPPLYLAETVSLLEEWGPPSSCPMQCKLTSHPARLTHLPPCLWGFAVALKPSWAGLAPSLLPPPRMSLCRPLSFLRHQCPWLPWQAHQGLVPWSPSMVAAACIVSPSGHCRCQPFIPHVFLGHGGLTSVSGECG

SEQ ID NO: 94 - protein, 259 aa, Homo sapiens
MAASRLELNLVRLLSRCEAMAAEKRDPDEWRLEKYVGALEDMLQALKVHASKPASEVINEYSWKVDFLKGMLQAEKLTSSSEKALANQFLAPGRVPTTARERVPATKTVHLQSRARYTSEMRSELLGTDSAEPEMDVRKRTGVAGSQPVSEKQLAAELDLVLQRHQNLQEKLAEEMLGLARSLKTNTLAAQSVIKKDNQTLSHSLKMADQNLEKLKTESERLEQHTQKSVNWLLWAMLIIVCFIFISMILFIRIMPKLK

SEQ ID NO: 95 - DNA, 1161 bp, synthetic construct
  source 1..1161: mol_type = other DNA
atgggctctatcggagccgccagcatggaattttgcttcgacgtgttcaaagagctgaaggtccaccacgccaacgagaacatcttctactgccctatcgccatcatgagcgccctggccatggtgtatctgggcgccaaggatagcacccggacacagatcaacaaggtcgtcagattcgacaagctgcccggcttcggcgattctatcgaagcccagtgtggcaccagcgtgaacgtgcacagcagcctgagagacatcctgaaccagatcaccaagcctaacgacgtgtacagcttcagcctggccagcagactgtacgccgaggaaagataccccatcctgcctgagtacctgcagtgcgtgaaagagctgtacagaggcggcctggaacctatcaacttccagacagccgccgaccaggccagagagctgatcaattcttgggtcgagagccagaccaacggcatcatcagaaacgtgctgcagcccagctccgtggattctcagacagccatggtgctggtcaacgccatcgtgtttaaaggcctgtgggagaaaaccttcaaggacgaggacacccaggccatgcctttcagagtgaccgagcaagagtccaagcctgtgcagatgatgtaccagatcggcctgtttagagtggcctccatggcctccgagaagatgaagatcctggaactgcctttcgccagcggcaccatgtctatgctggtgctgctgcctgatgaggtgtccggactggaacagctggaatccatcatcaacttcgagaagctgaccgagtggaccagcagcaacgtgatggaagaacggaagatcaaggtgtacctgcctcggatgaagatggaagagaagtacaacctgaccagcgtgctgatggccatgggaatcaccgatgtgttcagcagcagcgccaacctgagcggcattagctctgccgagagcctgaagattagccaggccgtgcatgctgcccacgccgagatcaatgaagccggcagagaagttgtgggatctgccgaagcaggcgtggacgctgcttctgtgtctgaggaattccgggccgaccatccttttctgttctgcatcaagcacattgccaccaacgccgtgctgttctttggcagatgcgtgtccccttga

SEQ ID NO: 96 - protein, 4 aa, synthetic construct
  REGION >4: note = The entire sequences of amino acids 1-4 can be repeated one to five times.
GGGS

SEQ ID NO: 97 - protein, 5 aa, synthetic construct
  REGION >5: note = The entire sequences of amino acids 1-5 can be repeated one to five times.
GGGGS

SEQ ID NO: 98 - protein, 5 aa, synthetic construct
  REGION >5: note = The entire sequences of amino acids 1-5 can be repeated one to five times.
EAAAK